European Patent Application EP 4 534 551 A1, published April 9, 2025. Title: Levadura y plásmido para la exposición de proteínas en superficie. Applicant: Universitat Politecnica de Valencia. The sequence listing filed with the application follows.

SEQUENCE LISTING (40 sequences)

SEQ ID NO: 1 - DNA, 644 bp, synthetic construct
  misc_feature 1..644: note = galactose-inducible promoter; note (original language) = Promotor inducible por galactosa
  source 1..644: mol_type = other DNA; organism (original language) = Secuencia artificial
tcattatcaatactcgccatttcaaagaatacgtaaataattaatagtagtgattttcctaactttatttagtcaaaaaattagccttttaattctgctgtaacccgtacatgcccaaaatagggggcgggttacacagaatatataacatcgtaggtgtctgggtgaacagtttattcctggcatccactaaatataatggagcccgctttttaagctggcatccagaaaaaaaaagaatcccagcaccaaaatattgttttcttcaccaaccatcagttcataggtccattctcttagcgcaactacagagaacaggggcacaaacaggcaaaaaacgggcacaacctcaatggagtgatgcaacctgcctggagtaaatgatgacacaaggcaattgacccacgcatgtatctatctcattttcttacaccttctattaccttctgctctctctgatttggaaaaagctgaaaaaaaaggttgaaaccagttccctgaaattattcccctacttgactaataagtatataaagacggtaggtattgattgtaattctgtaaatctatttcttaaacttcttaaattctacttttatagttagtcttttttttagttttaaaacaccagaacttagtttcga

SEQ ID NO: 2 - DNA, 6488 bp, synthetic construct
  misc_feature 1..6488: note = Plasmid PW22; note (original language) = Plásmido PW22
  source 1..6488: mol_type = other DNA
cggattagaagccgccgagcgggtgacagccctccgaaggaagactctcctccgtgcgtcctcgtcttcaccggtcgcgttcctgaaacgcagatgtgcctcgcgccgcactgctccgaacaataaagattctacaatactagcttttatggttatgaagaggaaaaattggcagtaacctggccccacaaaccttcaaatgaacgaatcaaattaacaaccataggatgataatgcgattagttttttagccttatttctggggtaattaatcagcgaagcgatgatttttgatctattaacagatatataaatgcaaaaactgcataaccactttaactaatactttcaacattttcggtttgtattacttcttattcaaatgtaataaaagtatcaacaaaaaattgttaatatacctctatactttaacgtcaaggagaaaaaaccccggatcgaattccctacttcatacattttcaattaagatgcagttacttcgctgtttttcaatattttctgttattgcttcagttttagcacaggaactgacaactatatgcgagcaaatcccctcaccaactttagaatcgacgccgtactctttgtcaacgactactattttggccaacgggaaggcaatgcaaggagtttttgaatattacaaatcagtaacgtttgtcagtaattgcggttctcacccctcaacaactagcaaaggcagccccataaacacacagtatgtttttaaggacaatagctcgacgattgaaggtagatacccatacgacgttccagactacgctctgcaggctagtggtggaggaggctctggtggaggcggtagcggaggcggagggtcggctagctgcggtggcggcggtactagcaaaatttctcattttttgaaaatggaatctttgaattttattagagctcatactccatatattaatatttacaattgtgaaccagctaatccatctgaaaaaaattctccatctactcaatattgttattctattcaatcttcccaggtcgactgcgggggcggatccgaacaaaagcttatttctgaagaggacttgtaatagctcgagatctgataacaacagtgtagatgtaacaaaatcgactttgttcccactgtacttttagctcgtacaaaatacaatatacttttcatttctccgtaaacaacatgttttcccatgtaatatccttttctatttttcgttccgttaccaactttacacatactttatatagctattcacttctatacactaaaaaactaagacaattttaattttgctgcctgccatatttcaatttgttataaattcctataatttatcctattagtagctaaaaaaagatgaatgtgaatcgaatcctaagagaattgagctccaattcgccctatagtgagtcgtattacaattcactggccgtcgttttacaacgtcgtgactgggaaaaccctggcgttacccaacttaatcgccttgcagcacatccccctttcgccagctggcgtaatagcgaagaggcccgcaccgatcgcctttcccaacagttgcgcagcctgaatggcgaatggacgcgccctgtagcggcgcattaagcgcggcgggtgtggtggttacgcgcagcgtgaccgctacacttgccagcgccctagcgcccgctcctttcgctttcttcccttcctttctcgccacgttcgccggctttccccgtcaagctctaaatcgggggctccctttagggttccgatttagtgctttacggcacctcgaccccaaaaaacttgattagggtgatggttcacgtagtgggccatcgccctgatagacggtttttcgccctttgacgttggagtccacgttctttaatagtggactcttgttccaaactggaacaacactcaaccctatctcggtctattcttttgatttataagggattttgccgatttcggcctattggttaaaaaatgagctgatttaacaaaaatttaacgcgaattttaacaaaatattaacgtttacaatttcctgatgcggtattttctccttacgcatctgtgcggtatttcacaccgcatagatccgtcgagttcaagagaaaaaaaaagaaaaagcaaaaagaaaaaaggaaagcgcgcctcgttcagaatgacacgtatagaatgatgcattaccttgtcatcttcagtatcatactgttcgtatacatacttactgacattcataggtatacatatatacacatgtatatatatcgtatgctgcagctttaaataatcggtgtcactacataagaacacctttggtggagggaacatcgttggtaccattgggcgaggtggcttctcttatggcaaccgcaagagccttgaacgcactctcactacggtgatgatcattcttgcctcgcagacaatcaacgtggagggtaattctgctagcctctgcaaagctttcaagaaaatgcgggatcatctcgcaagagagatctcctactttctccctttgcaaaccaagttcgacaactgcgtacggcctgttcgaaagatctaccaccgctctggaaagtgcctcatccaaaggcgcaaatcctgatccaaacctttttactccacgcgccagtagggcctctttaaaagcttgaccgagagcaatcccgcagtcttcagtggtgtgatggtcgtctatgtgtaagtcaccaatgcactcaacgattagcgaccagccggaatgcttggccagagcatgtatcatatggtccagaaaccctatacctgtgtggacgttaatcacttgcgattgtgtggcctgttctgctactgcttctgcctctttttctgggaagatcgagtgctctatcgctaggggaccaccctttaaagagatcgcaatctgaatcttggtttcatttgtaatacgctttactagggctttctgctctgtcatctttgccttcgtttatcttgcctgctcattttttagtatattcttcgaagaaatcacattactttatataatgtataattcattatgtgataatgccaatcgctaagaaaaaaaaagagtcatccgctaggggaaaaaaaaaaatgaaaatcattaccgaggcataaaaaaatatagagtgtactagaggaggccaagagtaatagaaaaagaaaattgcgggaaaggactgtgttatgacttccctgactaatgccgtgttcaaacgatacctggcagtgactcctagcgctcaccaagctcttaaaacgggaatttatggtgcactctcagtacaatctgctctgatgccgcatagttaagccagccccgacacccgccaacacccgctgacgcgccctgacgggcttgtctgctcccggcatccgcttacagacaagctgtgaccgtctccgggagctgcatgtgtcagaggttttcaccgtcatcaccgaaacgcgcgagacgaaagggcctcgtgatacgcctatttttataggttaatgtcatgataataatggtttcttagacggatcgcttgcctgtaacttacacgcgcctcgtatcttttaatgatggaataatttgggaatttactctgtgtttatttatttttatgttttgtatttggattttagaaagtaaataaagaaggtagaagagttacggaatgaagaaaaaaaaataaacaaaggtttaaaaaatttcaacaaaaagcgtactttacatatatatttattagacaagaaaagcagattaaatagatatacattcgattaacgataagtaaaatgtaaaatcacaggattttcgtgtgtggtcttctacacagacaagatgaaacaattcggcattaatacctgagagcaggaagagcaagataaaaggtagtatttgttggcgatccccctagagtcttttacatcttcggaaaacaaaaactattttttctttaatttctttttttactttctatttttaatttatatatttatattaaaaaatttaaattataattatttttatagcacgtgatgaaaaggacccaggtggcacttttcggggaaatgtgcgcggaacccctatttgtttatttttctaaatacattcaaatatgtatccgctcatgagacaataaccctgataaatgcttcaataatattgaaaaaggaagagtatgagtattcaacatttccgtgtcgcccttattcccttttttgcggcattttgccttcctgtttttgctcacccagaaacgctggtgaaagtaaaagatgctgaagatcagttgggtgcacgagtgggttacatcgaactggatctcaacagcggtaagatccttgagagttttcgccccgaagaacgttttccaatgatgagcacttttaaagttctgctatgtggcgcggtattatcccgtattgacgccgggcaagagcaactcggtcgccgcatacactattctcagaatgacttggttgagtactcaccagtcacagaaaagcatcttacggatggcatgacagtaagagaattatgcagtgctgccataaccatgagtgataacactgcggccaacttacttctgacaacgatcggaggaccgaaggagctaaccgcttttttgcacaacatgggggatcatgtaactcgccttgatcgttgggaaccggagctgaatgaagccataccaaacgacgagcgtgacaccacgatgcctgtagcaatggcaacaacgttgcgcaaactattaactggcgaactacttactctagcttcccggcaacaattaatagactggatggaggcggataaagttgcaggaccacttctgcgctcggcccttccggctggctggtttattgctgataaatctggagccggtgagcgtgggtctcgcggtatcattgcagcactggggccagatggtaagccctcccgtatcgtagttatctacacgacggggagtcaggcaactatggatgaacgaaatagacagatcgctgagataggtgcctcactgattaagcattggtaactgtcagaccaagtttactcatatatactttagattgatttaaaacttcatttttaatttaaaaggatctaggtgaagatcctttttgataatctcatgaccaaaatcccttaacgtgagttttcgttccactgagcgtcagaccccgtagaaaagatcaaaggatcttcttgagatcctttttttctgcgcgtaatctgctgcttgcaaacaaaaaaaccaccgctaccagcggtggtttgtttgccggatcaagagctaccaactctttttccgaaggtaactggcttcagcagagcgcagataccaaatactgttcttctagtgtagccgtagttaggccaccacttcaagaactctgtagcaccgcctacatacctcgctctgctaatcctgttaccagtggctgctgccagtggcgataagtcgtgtcttaccgggttggactcaagacgatagttaccggataaggcgcagcggtcgggctgaacggggggttcgtgcacacagcccagcttggagcgaacgacctacaccgaactgagatacctacagcgtgagctatgagaaagcgccacgcttcccgaagggagaaaggcggacaggtatccggtaagcggcagggtcggaacaggagagcgcacgagggagcttccagggggaaacgcctggtatctttatagtcctgtcgggtttcgccacctctgacttgagcgtcgatttttgtgatgctcgtcaggggggcggagcctatggaaaaacgccagcaacgcggcctttttacggttcctggccttttgctggccttttgctcacatgttctttcctgcgttatcccctgattctgtggataaccgtattaccgcctttgagtgagctgataccgctcgccgcagccgaacgaccgagcgcagcgagtcagtgagcgaggaagcggaagagcgcccaatacgcaaaccgcctctccccgcgcgttggccgattcattaatgcagctggcacgacaggtttcccgactggaaagcgggcagtgagcgcaacgcaattaatgtgagttagctcactcattaggcaccccaggctttacactttatgcttccggctcgtatgttgtgtggaattgtgagcggataacaatttcacacaggaaacagctatgaccatgattacgccaagctcgaaattaaccctcactaaagggaacaaaagctggtaccaattccttgaattttcaaaaattcttactttttttttggatggacgcaaagaagtttaataatcatattacatggcattaccaccatatacatatccatatctaatcttacttatatgttgtggaaatgtaaagagccccattatcttagcctaaaaaaaccttctctttggaactttcagtaatacgcttaactgctcattgctatattgaagta

SEQ ID NO: 3 - DNA, 7532 bp, synthetic construct
  misc_feature 1..7532: note = Plasmid PW23; note (original language) = Plásmido PW23
  source 1..7532: mol_type = other DNA
cggattagaagccgccgagcgggtgacagccctccgaaggaagactctcctccgtgcgtcctcgtcttcaccggtcgcgttcctgaaacgcagatgtgcctcgcgccgcactgctccgaacaataaagattctacaatactagcttttatggttatgaagaggaaaaattggcagtaacctggccccacaaaccttcaaatgaacgaatcaaattaacaaccataggatgataatgcgattagttttttagccttatttctggggtaattaatcagcgaagcgatgatttttgatctattaacagatatataaatgcaaaaactgcataaccactttaactaatactttcaacattttcggtttgtattacttcttattcaaatgtaataaaagtatcaacaaaaaattgttaatatacctctatactttaacgtcaaggagaaaaaaccccggatcgaattccctacttcatacattttcaattaagatgcagttacttcgctgtttttcaatattttctgttattgcttcagttttagcacaggaactgacaactatatgcgagcaaatcccctcaccaactttagaatcgacgccgtactctttgtcaacgactactattttggccaacgggaaggcaatgcaaggagtttttgaatattacaaatcagtaacgtttgtcagtaattgcggttctcacccctcaacaactagcaaaggcagccccataaacacacagtatgtttttaaggacaatagctcgacgattgaaggtagatacccatacgacgttccagactacgctctgcaggctagtggtggaggaggctctggtggaggcggtagcggaggcggagggtcggctagctgcggtggcggcggtactagcaaaatttctcattttttgaaaatggaatctttgaattttattagagctcatactccatatattaatatttacaattgtgaaccagctaatccatctgaaaaaaattctccatctactcaatattgttattctattcaatcttcccaggtcgactgcgggggcggatccgaacaaaagcttatttctgaagaggacttgtaatagctcgagatctgataacaacagtgtagatgtaacaaaatcgactttgttcccactgtacttttagctcgtacaaaatacaatatacttttcatttctccgtaaacaacatgttttcccatgtaatatccttttctatttttcgttccgttaccaactttacacatactttatatagctattcacttctatacactaaaaaactaagacaattttaattttgctgcctgccatatttcaatttgttataaattcctataatttatcctattagtagctaaaaaaagatgaatgtgaatcgaatcctaagagaattgagctccaattcgccctatagtgagtcgtattacaattcactggccgtcgttttacaacgtcgtgactgggaaaaccctggcgttacccaacttaatcgccttgcagcacatccccctttcgccagctggcgtaatagcgaagaggcccgcaccgatcgcctttcccaacagttgcgcagcctgaatggcgaatggacgcgccctgtagcggcgcattaagcgcggcgggtgtggtggttacgcgcagcgtgaccgctacacttgccagcgccctagcgcccgctcctttcgctttcttcccttcctttctcgccacgttcgccggctttccccgtcaagctctaaatcgggggctccctttagggttccgatttagtgctttacggcacctcgaccccaaaaaacttgattagggtgatggttcacgtagtgggccatcgccctgatagacggtttttcgccctttgacgttggagtccacgttctttaatagtggactcttgttccaaactggaacaacactcaaccctatctcggtctattcttttgatttataagggattttgccgatttcggcctattggttaaaaaatgagctgatttaacaaaaatttaacgcgaattttaacaaaatattaacgcttacaatttcctgatgcggtattttctccttacgcatctgtgcggtatttcacaccgcatatcgaccggtcgaggagaacttctagtatatctacatacctaatattattgccttattaaaaatggaatcccaacaattacatcaaaatccacattctcttcaaaatcaattgtcctgtacttccttgttcatgtgtgttcaaaaacgttatatttataggataattatactctatttctcaacaagtaattggttgtttggccgagcggtctaaggcgcctgattcaagaaatatcttgaccgcagttaactgtgggaatactcaggtatcgtaagatgcaagagttcgaatctcttagcaaccattatttttttcctcaacataacgagaacacacaggggcgctatcgcacagaatcaaattcgatgactggaaattttttgttaatttcagaggtcgcctgacgcatatacctttttcaactgaaaaattgggagaaaaaggaaaggtgagagcgccggaaccggcttttcatatagaatagagaagcgttcatgactaaatgcttgcatcacaatacttgaagttgacaatattatttaaggacctattgttttttccaataggtggttagcaatcgtcttactttctaacttttcttaccttttacatttcagcaatatatatatatatatttcaaggatataccattctaatgtctgcccctaagaagatcgtcgttttgccaggtgaccacgttggtcaagaaatcacagccgaagccattaaggttcttaaagctatttctgatgttcgttccaatgtcaagttcgatttcgaaaatcatttaattggtggtgctgctatcgatgctacaggtgttccacttccagatgaggcgctggaagcctccaagaaggctgatgccgttttgttaggtgctgtgggtggtcctaaatggggtaccggtagtgttagacctgaacaaggtttactaaaaatccgtaaagaacttcaattgtacgccaacttaagaccatgtaactttgcatccgactctcttttagacttatctccaatcaagccacaatttgctaaaggtactgacttcgttgttgtcagagaattagtgggaggtatttactttggtaagagaaaggaagacgatggtgatggtgtcgcttgggatagtgaacaatacaccgttccagaagtgcaaagaatcacaagaatggccgctttcatggccctacaacatgagccaccattgcctatttggtccttggataaagctaatgttttggcctcttcaagattatggagaaaaactgtggaggaaaccatcaagaacgaattccctacattgaaggttcaacatcaattgattgattctgccgccatgatcctagttaagaacccaacccacctaaatggtattataatcaccagcaacatgtttggtgatatcatctccgatgaagcctccgttatcccaggttccttgggtttgttgccatctgcgtccttggcctctttgccagacaagaacaccgcatttggtttgtacgaaccatgccacggttctgctccagatttgccaaagaataaggtcaaccctatcgccactatcttgtctgctgcaatgatgttgaaattgtcattgaacttgcctgaagaaggtaaggccattgaagatgcagttaaaaaggttttggatgcaggtatcagaactggtgatttaggtggttccaacagtaccaccgaagtcggtgatgctgtcgccgaagaagttaagaaaatccttgcttaaaaagattctctttttttatgatatttgtacataaactttataaatgaaattcataatagaaacgacacgaaattacaaaatggaatatgttcatagggtagacgaaactatatacgcaatctacatacatttatcaagaaggagaaaaaggaggatgtaaaggaatacaggtaagcaaattgatactaatggctcaacgtgataaggaaaaagaattgcactttaacattaatattgacaaggaggagggcaccacacaaaaagttaggtgtaacagaaaatcatgaaactatgattcctaatttatatattggaggattttctctaaaaaaaaaaaaatacaacaaataaaaaacactcaatgacctgaccatttgatggagtttaagtcaataccttcttgaaccatttcccataatggtgaaagttccctcaagaattttactctgtcagaaacggccttaacgacgtagtcgatatggtgcactctcagtacaatctgctctgatgccgcatagttaagccagccccgacacccgccaacacccgctgacgcgccctgacgggcttgtctgctcccggcatccgcttacagacaagctgtgaccgtctccgggagctgcatgtgtcagaggttttcaccgtcatcaccgaaacgcgcgagacgaaagggcctcgtgatacgcctatttttataggttaatgtcatgataataatggtttcttagacggatcgcttgcctgtaacttacacgcgcctcgtatcttttaatgatggaataatttgggaatttactctgtgtttatttatttttatgttttgtatttggattttagaaagtaaataaagaaggtagaagagttacggaatgaagaaaaaaaaataaacaaaggtttaaaaaatttcaacaaaaagcgtactttacatatatatttattagacaagaaaagcagattaaatagatatacattcgattaacgataagtaaaatgtaaaatcacaggattttcgtgtgtggtcttctacacagacaagatgaaacaattcggcattaatacctgagagcaggaagagcaagataaaaggtagtatttgttggcgatccccctagagtcttttacatcttcggaaaacaaaaactattttttctttaatttctttttttactttctatttttaatttatatatttatattaaaaaatttaaattataattatttttatagcacgtgatgaaaaggacccaggtggcacttttcggggaaatgtgcgcggaacccctatttgtttatttttctaaatacattcaaatatgtatccgctcatgagacaataaccctgataaatgcttcaataatattgaaaaaggaagagtatgagtattcaacatttccgtgtcgcccttattcccttttttgcggcattttgccttcctgtttttgctcacccagaaacgctggtgaaagtaaaagatgctgaagatcagttgggtgcacgagtgggttacatcgaactggatctcaacagcggtaagatccttgagagttttcgccccgaagaacgttttccaatgatgagcacttttaaagttctgctatgtggcgcggtattatcccgtattgacgccgggcaagagcaactcggtcgccgcatacactattctcagaatgacttggttgagtactcaccagtcacagaaaagcatcttacggatggcatgacagtaagagaattatgcagtgctgccataaccatgagtgataacactgcggccaacttacttctgacaacgatcggaggaccgaaggagctaaccgcttttttgcacaacatgggggatcatgtaactcgccttgatcgttgggaaccggagctgaatgaagccataccaaacgacgagcgtgacaccacgatgcctgtagcaatggcaacaacgttgcgcaaactattaactggcgaactacttactctagcttcccggcaacaattaatagactggatggaggcggataaagttgcaggaccacttctgcgctcggcccttccggctggctggtttattgctgataaatctggagccggtgagcgtgggtctcgcggtatcattgcagcactggggccagatggtaagccctcccgtatcgtagttatctacacgacggggagtcaggcaactatggatgaacgaaatagacagatcgctgagataggtgcctcactgattaagcattggtaactgtcagaccaagtttactcatatatactttagattgatttaaaacttcatttttaatttaaaaggatctaggtgaagatcctttttgataatctcatgaccaaaatcccttaacgtgagttttcgttccactgagcgtcagaccccgtagaaaagatcaaaggatcttcttgagatcctttttttctgcgcgtaatctgctgcttgcaaacaaaaaaaccaccgctaccagcggtggtttgtttgccggatcaagagctaccaactctttttccgaaggtaactggcttcagcagagcgcagataccaaatactgttcttctagtgtagccgtagttaggccaccacttcaagaactctgtagcaccgcctacatacctcgctctgctaatcctgttaccagtggctgctgccagtggcgataagtcgtgtcttaccgggttggactcaagacgatagttaccggataaggcgcagcggtcgggctgaacggggggttcgtgcacacagcccagcttggagcgaacgacctacaccgaactgagatacctacagcgtgagctatgagaaagcgccacgcttcccgaagggagaaaggcggacaggtatccggtaagcggcagggtcggaacaggagagcgcacgagggagcttccagggggaaacgcctggtatctttatagtcctgtcgggtttcgccacctctgacttgagcgtcgatttttgtgatgctcgtcaggggggcggagcctatggaaaaacgccagcaacgcggcctttttacggttcctggccttttgctggccttttgctcacatgttctttcctgcgttatcccctgattctgtggataaccgtattaccgcctttgagtgagctgataccgctcgccgcagccgaacgaccgagcgcagcgagtcagtgagcgaggaagcggaagagcgcccaatacgcaaaccgcctctccccgcgcgttggccgattcattaatgcagctggcacgacaggtttcccgactggaaagcgggcagtgagcgcaacgcaattaatgtgagttagctcactcattaggcaccccaggctttacactttatgcttccggctcgtatgttgtgtggaattgtgagcggataacaatttcacacaggaaacagctatgaccatgattacgccaagctcgaaattaaccctcactaaagggaacaaaagctggtaccaattccttgaattttcaaaaattcttactttttttttggatggacgcaaagaagtttaataatcatattacatggcattaccaccatatacatatccatatctaatcttacttatatgttgtggaaatgtaaagagccccattatcttagcctaaaaaaaccttctctttggaactttcagtaatacgcttaactgctcattgctatattgaagta

SEQ ID NO: 4 - DNA, 6341 bp, synthetic construct
  misc_feature 1..6341: note = Plasmid PW24; note (original language) = Plásmido PW24
  source 1..6341: mol_type = other DNA
cggattagaagccgccgagcgggtgacagccctccgaaggaagactctcctccgtgcgtcctcgtcttcaccggtcgcgttcctgaaacgcagatgtgcctcgcgccgcactgctccgaacaataaagattctacaatactagcttttatggttatgaagaggaaaaattggcagtaacctggccccacaaaccttcaaatgaacgaatcaaattaacaaccataggatgataatgcgattagttttttagccttatttctggggtaattaatcagcgaagcgatgatttttgatctattaacagatatataaatgcaaaaactgcataaccactttaactaatactttcaacattttcggtttgtattacttcttattcaaatgtaataaaagtatcaacaaaaaattgttaatatacctctatactttaacgtcaaggagaaaaaaccccggatcgaattccctacttcatacattttcaattaagatgcagttacttcgctgtttttcaatattttctgttattgcttcagttttagcacaggaactgacaactatatgcgagcaaatcccctcaccaactttagaatcgacgccgtactctttgtcaacgactactattttggccaacgggaaggcaatgcaaggagtttttgaatattacaaatcagtaacgtttgtcagtaattgcggttctcacccctcaacaactagcaaaggcagccccataaacacacagtatgtttttaaggacaatagctcgacgattgaaggtagatacccatacgacgttccagactacgctctgcaggaaaatttgtattttcaatctctgcaggctagtggtggaggaggctctggtggaggcggtagcggaggcggagggtcggctagctgcggtggcggcggtactagcaaaatttctcattttttgaaaatggaatctttgaattttattagagctcatactccatatattaatatttacaattgtgaaccagctaatccatctgaaaaaaattctccatctactcaatattgttattctattcaatcttcccaggtcgactgcgggggcggatccgaacaaaagcttatttctgaagaggacttgtaatagctcgagatctgataacaacagtgtagatgtaacaaaatcgactttgttcccactgtacttttagctcgtacaaaatacaatatacttttcatttctccgtaaacaacatgttttcccatgtaatatccttttctatttttcgttccgttaccaactttacacatactttatatagctattcacttctatacactaaaaaactaagacaattttaattttgctgcctgccatatttcaatttgttataaattcctataatttatcctattagtagctaaaaaaagatgaatgtgaatcgaatcctaagagaattgagctccaattcgccctatagtgagtcgtattacaattcactggccgtcgttttacaacgtcgtgactgggaaaaccctggcgttacccaacttaatcgccttgcagcacatccccctttcgccagctggcgtaatagcgaagaggcccgcaccgatcgcctttcccaacagttgcgcagcctgaatggcgaatggacgcgccctgtagcggcgcattaagcgcggcgggtgtggtggttacgcgcagcgtgaccgctacacttgccagcgccctagcgcccgctcctttcgctttcttcccttcctttctcgccacgttcgccggctttccccgtcaagctctaaatcgggggctccctttagggttccgatttagtgctttacggcacctcgaccccaaaaaacttgattagggtgatggttcacgtagtgggccatcgccctgatagacggtttttcgccctttgacgttggagtccacgttctttaatagtggactcttgttccaaactggaacaacactcaaccctatctcggtctattcttttgatttataagggattttgccgatttcggcctattggttaaaaaatgagctgatttaacaaaaatttaacgcgaattttaacaaaatattaacgcttacaatttcctgatgcggtattttctccttacgcatctgtgcggtatttcacaccgcatagatcggcaagtgcacaaacaatacttaaataaatactactcagtaataacctatttcttagcatttttgacgaaatttgctattttgttagagtcttttacaccatttgtctccacacctccgcttacatcaacaccaataacgccatttaatctaagcgcatcaccaacattttctggcgtcagtccaccagctaacataaaatgtaagctttcggggctctcttgccttccaacccagtcagaaatcgagttccaatccaaaagttcacctgtcccacctgcttctgaatcaaacaagggaataaacgaatgaggtttctgtgaagctgcactgagtagtatgttgcagtcttttggaaatacgagtcttttaataactggcaaaccgaggaactcttggtattcttgccacgactcatctccatgcagttggacgatatcaatgccgtaatcattgaccagagccaaaacatcctccttaggttgattacgaaacacgccaaccaagtatttcggagtgcctgaactatttttatatgcttttacaagacttgaaattttccttgcaataaccgggtcaattgttctctttctattgggcacacatataatacccagcaagtcagcatcggaatctagagcacattctgcggcctctgtgctctgcaagccgcaaactttcaccaatggaccagaactacctgtgaaattaataacagacatactccaagctgcctttgtgtgcttaatcacgtatactcacgtgctcaatagtcaccaatgccctccctcttggccctctccttttcttttttcgaccgaattaattcttaatcggcaaaaaaagaaaagctccggatcaagattgtacgtaaggtgacaagctatttttcaataaagaatatcttccactactgccatctggcgtcataactgcaaagtacacatatattacgatgctgttctattaaatgcttcctatattatatatatagtaatgtcgtgatctatggtgcactctcagtacaatctgctctgatgccgcatagttaagccagccccgacacccgccaacacccgctgacgcgccctgacgggcttgtctgctcccggcatccgcttacagacaagctgtgaccgtctccgggagctgcatgtgtcagaggttttcaccgtcatcaccgaaacgcgcgagacgaaagggcctcgtgatacgcctatttttataggttaatgtcatgataataatggtttcttagacggatcgcttgcctgtaacttacacgcgcctcgtatcttttaatgatggaataatttgggaatttactctgtgtttatttatttttatgttttgtatttggattttagaaagtaaataaagaaggtagaagagttacggaatgaagaaaaaaaaataaacaaaggtttaaaaaatttcaacaaaaagcgtactttacatatatatttattagacaagaaaagcagattaaatagatatacattcgattaacgataagtaaaatgtaaaatcacaggattttcgtgtgtggtcttctacacagacaagatgaaacaattcggcattaatacctgagagcaggaagagcaagataaaaggtagtatttgttggcgatccccctagagtcttttacatcttcggaaaacaaaaactattttttctttaatttctttttttactttctatttttaatttatatatttatattaaaaaatttaaattataattatttttatagcacgtgatgaaaaggacccaggtggcacttttcggggaaatgtgcgcggaacccctatttgtttatttttctaaatacattcaaatatgtatccgctcatgagacaataaccctgataaatgcttcaataatattgaaaaaggaagagtatgagtattcaacatttccgtgtcgcccttattcccttttttgcggcattttgccttcctgtttttgctcacccagaaacgctggtgaaagtaaaagatgctgaagatcagttgggtgcacgagtgggttacatcgaactggatctcaacagcggtaagatccttgagagttttcgccccgaagaacgttttccaatgatgagcacttttaaagttctgctatgtggcgcggtattatcccgtattgacgccgggcaagagcaactcggtcgccgcatacactattctcagaatgacttggttgagtactcaccagtcacagaaaagcatcttacggatggcatgacagtaagagaattatgcagtgctgccataaccatgagtgataacactgcggccaacttacttctgacaacgatcggaggaccgaaggagctaaccgcttttttgcacaacatgggggatcatgtaactcgccttgatcgttgggaaccggagctgaatgaagccataccaaacgacgagcgtgacaccacgatgcctgtagcaatggcaacaacgttgcgcaaactattaactggcgaactacttactctagcttcccggcaacaattaatagactggatggaggcggataaagttgcaggaccacttctgcgctcggcccttccggctggctggtttattgctgataaatctggagccggtgagcgtgggtctcgcggtatcattgcagcactggggccagatggtaagccctcccgtatcgtagttatctacacgacggggagtcaggcaactatggatgaacgaaatagacagatcgctgagataggtgcctcactgattaagcattggtaactgtcagaccaagtttactcatatatactttagattgatttaaaacttcatttttaatttaaaaggatctaggtgaagatcctttttgataatctcatgaccaaaatcccttaacgtgagttttcgttccactgagcgtcagaccccgtagaaaagatcaaaggatcttcttgagatcctttttttctgcgcgtaatctgctgcttgcaaacaaaaaaaccaccgctaccagcggtggtttgtttgccggatcaagagctaccaactctttttccgaaggtaactggcttcagcagagcgcagataccaaatactgttcttctagtgtagccgtagttaggccaccacttcaagaactctgtagcaccgcctacatacctcgctctgctaatcctgttaccagtggctgctgccagtggcgataagtcgtgtcttaccgggttggactcaagacgatagttaccggataaggcgcagcggtcgggctgaacggggggttcgtgcacacagcccagcttggagcgaacgacctacaccgaactgagatacctacagcgtgagctatgagaaagcgccacgcttcccgaagggagaaaggcggacaggtatccggtaagcggcagggtcggaacaggagagcgcacgagggagcttccagggggaaacgcctggtatctttatagtcctgtcgggtttcgccacctctgacttgagcgtcgatttttgtgatgctcgtcaggggggcggagcctatggaaaaacgccagcaacgcggcctttttacggttcctggccttttgctggccttttgctcacatgttctttcctgcgttatcccctgattctgtggataaccgtattaccgcctttgagtgagctgataccgctcgccgcagccgaacgaccgagcgcagcgagtcagtgagcgaggaagcggaagagcgcccaatacgcaaaccgcctctccccgcgcgttggccgattcattaatgcagctggcacgacaggtttcccgactggaaagcgggcagtgagcgcaacgcaattaatgtgagttagctcactcattaggcaccccaggctttacactttatgcttccggctcgtatgttgtgtggaattgtgagcggataacaatttcacacaggaaacagctatgaccatgattacgccaagctcgaaattaaccctcactaaagggaacaaaagctggtaccaattccttgaattttcaaaaattcttactttttttttggatggacgcaaagaagtttaataatcatattacatggcattaccaccatatacatatccatatctaatcttacttatatgttgtggaaatgtaaagagccccattatcttagcctaaaaaaaccttctctttggaactttcagtaatacgcttaactgctcattgctatattgaagta

SEQ ID NO: 5 - DNA, 6515 bp, synthetic construct
  misc_feature 1..6515: note = Plasmid PW25; note (original language) = Plásmido PW25
  source 1..6515: mol_type = other DNA
cggattagaagccgccgagcgggtgacagccctccgaaggaagactctcctccgtgcgtcctcgtcttcaccggtcgcgttcctgaaacgcagatgtgcctcgcgccgcactgctccgaacaataaagattctacaatactagcttttatggttatgaagaggaaaaattggcagtaacctggccccacaaaccttcaaatgaacgaatcaaattaacaaccataggatgataatgcgattagttttttagccttatttctggggtaattaatcagcgaagcgatgatttttgatctattaacagatatataaatgcaaaaactgcataaccactttaactaatactttcaacattttcggtttgtattacttcttattcaaatgtaataaaagtatcaacaaaaaattgttaatatacctctatactttaacgtcaaggagaaaaaaccccggatcgaattccctacttcatacattttcaattaagatgcagttacttcgctgtttttcaatattttctgttattgcttcagttttagcacaggaactgacaactatatgcgagcaaatcccctcaccaactttagaatcgacgccgtactctttgtcaacgactactattttggccaacgggaaggcaatgcaaggagtttttgaatattacaaatcagtaacgtttgtcagtaattgcggttctcacccctcaacaactagcaaaggcagccccataaacacacagtatgtttttaaggacaatagctcgacgattgaaggtagatacccatacgacgttccagactacgctctgcaggaaaatttgtattttcaatctctgcaggctagtggtggaggaggctctggtggaggcggtagcggaggcggagggtcggctagctgcggtggcggcggtactagcaaaatttctcattttttgaaaatggaatctttgaattttattagagctcatactccatatattaatatttacaattgtgaaccagctaatccatctgaaaaaaattctccatctactcaatattgttattctattcaatcttcccaggtcgactgcgggggcggatccgaacaaaagcttatttctgaagaggacttgtaatagctcgagatctgataacaacagtgtagatgtaacaaaatcgactttgttcccactgtacttttagctcgtacaaaatacaatatacttttcatttctccgtaaacaacatgttttcccatgtaatatccttttctatttttcgttccgttaccaactttacacatactttatatagctattcacttctatacactaaaaaactaagacaattttaattttgctgcctgccatatttcaatttgttataaattcctataatttatcctattagtagctaaaaaaagatgaatgtgaatcgaatcctaagagaattgagctccaattcgccctatagtgagtcgtattacaattcactggccgtcgttttacaacgtcgtgactgggaaaaccctggcgttacccaacttaatcgccttgcagcacatccccctttcgccagctggcgtaatagcgaagaggcccgcaccgatcgcctttcccaacagttgcgcagcctgaatggcgaatggacgcgccctgtagcggcgcattaagcgcggcgggtgtggtggttacgcgcagcgtgaccgctacacttgccagcgccctagcgcccgctcctttcgctttcttcccttcctttctcgccacgttcgccggctttccccgtcaagctctaaatcgggggctccctttagggttccgatttagtgctttacggcacctcgaccccaaaaaacttgattagggtgatggttcacgtagtgggccatcgccctgatagacggtttttcgccctttgacgttggagtccacgttctttaatagtggactcttgttccaaactggaacaacactcaaccctatctcggtctattcttttgatttataagggattttgccgatttcggcctattggttaaaaaatgagctgatttaacaaaaatttaacgcgaattttaacaaaatattaacgtttacaatttcctgatgcggtattttctccttacgcatctgtgcggtatttcacaccgcatagatccgtcgagttcaagagaaaaaaaaagaaaaagcaaaaagaaaaaaggaaagcgcgcctcgttcagaatgacacgtatagaatgatgcattaccttgtcatcttcagtatcatactgttcgtatacatacttactgacattcataggtatacatatatacacatgtatatatatcgtatgctgcagctttaaataatcggtgtcactacataagaacacctttggtggagggaacatcgttggtaccattgggcgaggtggcttctcttatggcaaccgcaagagccttgaacgcactctcactacggtgatgatcattcttgcctcgcagacaatcaacgtggagggtaattctgctagcctctgcaaagctttcaagaaaatgcgggatcatctcgcaagagagatctcctactttctccctttgcaaaccaagttcgacaactgcgtacggcctgttcgaaagatctaccaccgctctggaaagtgcctcatccaaaggcgcaaatcctgatccaaacctttttactccacgcgccagtagggcctctttaaaagcttgaccgagagcaatcccgcagtcttcagtggtgtgatggtcgtctatgtgtaagtcaccaatgcactcaacgattagcgaccagccggaatgcttggccagagcatgtatcatatggtccagaaaccctatacctgtgtggacgttaatcacttgcgattgtgtggcctgttctgctactgcttctgcctctttttctgggaagatcgagtgctctatcgctaggggaccaccctttaaagagatcgcaatctgaatcttggtttcatttgtaatacgctttactagggctttctgctctgtcatctttgccttcgtttatcttgcctgctcattttttagtatattcttcgaagaaatcacattactttatataatgtataattcattatgtgataatgccaatcgctaagaaaaaaaaagagtcatccgctaggggaaaaaaaaaaatgaaaatcattaccgaggcataaaaaaatatagagtgtactagaggaggccaagagtaatagaaaaagaaaattgcgggaaaggactgtgttatgacttccctgactaatgccgtgttcaaacgatacctggcagtgactcctagcgctcaccaagctcttaaaacgggaatttatggtgcactctcagtacaatctgctctgatgccgcatagttaagccagccccgacacccgccaacacccgctgacgcgccctgacgggcttgtctgctcccggcatccgcttacagacaagctgtgaccgtctccgggagctgcatgtgtcagaggttttcaccgtcatcaccgaaacgcgcgagacgaaagggcctcgtgatacgcctatttttataggttaatgtcatgataataatggtttcttagacggatcgcttgcctgtaacttacacgcgcctcgtatcttttaatgatggaataatttgggaatttactctgtgtttatttatttttatgttttgtatttggattttagaaagtaaataaagaaggtagaagagttacggaatgaagaaaaaaaaataaacaaaggtttaaaaaatttcaacaaaaagcgtactttacatatatatttattagacaagaaaagcagattaaatagatatacattcgattaacgataagtaaaatgtaaaatcacaggattttcgtgtgtggtcttctacacagacaagatgaaacaattcggcattaatacctgagagcaggaagagcaagataaaaggtagtatttgttggcgatccccctagagtcttttacatcttcggaaaacaaaaactattttttctttaatttctttttttactttctatttttaatttatatatttatattaaaaaatttaaattataattatttttatagcacgtgatgaaaaggacccaggtggcacttttcggggaaatgtgcgcggaacccctatttgtttatttttctaaatacattcaaatatgtatccgctcatgagacaataaccctgataaatgcttcaataatattgaaaaaggaagagtatgagtattcaacatttccgtgtcgcccttattcccttttttgcggcattttgccttcctgtttttgctcacccagaaacgctggtgaaagtaaaagatgctgaagatcagttgggtgcacgagtgggttacatcgaactggatctcaacagcggtaagatccttgagagttttcgccccgaagaacgttttccaatgatgagcacttttaaagttctgctatgtggcgcggtattatcccgtattgacgccgggcaagagcaactcggtcgccgcatacactattctcagaatgacttggttgagtactcaccagtcacagaaaagcatcttacggatggcatgacagtaagagaattatgcagtgctgccataaccatgagtgataacactgcggccaacttacttctgacaacgatcggaggaccgaaggagctaaccgcttttttgcacaacatgggggatcatgtaactcgccttgatcgttgggaaccggagctgaatgaagccataccaaacgacgagcgtgacaccacgatgcctgtagcaatggcaacaacgttgcgcaaactattaactggcgaactacttactctagcttcccggcaacaattaatagactggatggaggcggataaagttgcaggaccacttctgcgctcggcccttccggctggctggtttattgctgataaatctggagccggtgagcgtgggtctcgcggtatcattgcagcactggggccagatggtaagccctcccgtatcgtagttatctacacgacggggagtcaggcaactatggatgaacgaaatagacagatcgctgagataggtgcctcactgattaagcattggtaactgtcagaccaagtttactcatatatactttagattgatttaaaacttcatttttaatttaaaaggatctaggtgaagatcctttttgataatctcatgaccaaaatcccttaacgtgagttttcgttccactgagcgtcagaccccgtagaaaagatcaaaggatcttcttgagatcctttttttctgcgcgtaatctgctgcttgcaaacaaaaaaaccaccgctaccagcggtggtttgtttgccggatcaagagctaccaactctttttccgaaggtaactggcttcagcagagcgcagataccaaatactgttcttctagtgtagccgtagttaggccaccacttcaagaactctgtagcaccgcctacatacctcgctctgctaatcctgttaccagtggctgctgccagtggcgataagtcgtgtcttaccgggttggactcaagacgatagttaccggataaggcgcagcggtcgggctgaacggggggttcgtgcacacagcccagcttggagcgaacgacctacaccgaactgagatacctacagcgtgagctatgagaaagcgccacgcttcccgaagggagaaaggcggacaggtatccggtaagcggcagggtcggaacaggagagcgcacgagggagcttccagggggaaacgcctggtatctttatagtcctgtcgggtttcgccacctctgacttgagcgtcgatttttgtgatgctcgtcaggggggcggagcctatggaaaaacgccagcaacgcggcctttttacggttcctggccttttgctggccttttgctcacatgttctttcctgcgttatcccctgattctgtggataaccgtattaccgcctttgagtgagctgataccgctcgccgcagccgaacgaccgagcgcagcgagtcagtgagcgaggaagcggaagagcgcccaatacgcaaaccgcctctccccgcgcgttggccgattcattaatgcagctggcacgacaggtttcccgactggaaagcgggcagtgagcgcaacgcaattaatgtgagttagctcactcattaggcaccccaggctttacactttatgcttccggctcgtatgttgtgtggaattgtgagcggataacaatttcacacaggaaacagctatgaccatgattacgccaagctcgaaattaaccctcactaaagggaacaaaagctggtaccaattccttgaattttcaaaaattcttactttttttttggatggacgcaaagaagtttaataatcatattacatggcattaccaccatatacatatccatatctaatcttacttatatgttgtggaaatgtaaagagccccattatcttagcctaaaaaaaccttctctttggaactttcagtaatacgcttaactgctcattgctatattgaagta

SEQ ID NO: 6 - DNA, 7559 bp, synthetic construct
  misc_feature 1..7559: note = Plasmid PW26; note (original language) = Plásmido PW26
  source 1..7559: mol_type = other DNA
cggattagaagccgccgagcgggtgacagccctccgaaggaagactctcctccgtgcgtcctcgtcttcaccggtcgcgttcctgaaacgcagatgtgcctcgcgccgcactgctccgaacaataaagattctacaatactagcttttatggttatgaagaggaaaaattggcagtaacctggccccacaaaccttcaaatgaacgaatcaaattaacaaccataggatgataatgcgattagttttttagccttatttctggggtaattaatcagcgaagcgatgatttttgatctattaacagatatataaatgcaaaaactgcataaccactttaactaatactttcaacattttcggtttgtattacttcttattcaaatgtaataaaagtatcaacaaaaaattgttaatatacctctatactttaacgtcaaggagaaaaaaccccggatcgaattccctacttcatacattttcaattaagatgcagttacttcgctgtttttcaatattttctgttattgcttcagttttagcacaggaactgacaactatatgcgagcaaatcccctcaccaactttagaatcgacgccgtactctttgtcaacgactactattttggccaacgggaaggcaatgcaaggagtttttgaatattacaaatcagtaacgtttgtcagtaattgcggttctcacccctcaacaactagcaaaggcagccccataaacacacagtatgtttttaaggacaatagctcgacgattgaaggtagatacccatacgacgttccagactacgctctgcaggaaaatttgtattttcaatctctgcaggctagtggtggaggaggctctggtggaggcggtagcggaggcggagggtcggctagctgcggtggcggcggtactagcaaaatttctcattttttgaaaatggaatctttgaattttattagagctcatactccatatattaatatttacaattgtgaaccagctaatccatctgaaaaaaattctccatctactcaatattgttattctattcaatcttcccaggtcgactgcgggggcggatccgaacaaaagcttatttctgaagaggacttgtaatagctcgagatctgataacaacagtgtagatgtaacaaaatcgactttgttcccactgtacttttagctcgtacaaaatacaatatacttttcatttctccgtaaacaacatgttttcccatgtaatatccttttctatttttcgttccgttaccaactttacacatactttatatagctattcacttctatacactaaaaaactaagacaattttaattttgctgcctgccatatttcaatttgttataaattcctataatttatcctattagtagctaaaaaaagatgaatgtgaatcgaatcctaagagaattgagctccaattcgccctatagtgagtcgtattacaattcactggccgtcgttttacaacgtcgtgactgggaaaaccctggcgttacccaacttaatcgccttgcagcacatccccctttcgccagctggcgtaatagcgaagaggcccgcaccgatcgcctttcccaacagttgcgcagcctgaatggcgaatggacgcgccctgtagcggcgcattaagcgcggcgggtgtggtggttacgcgcagcgtgaccgctacacttgccagcgccctagcgcccgctcctttcgctttcttcccttcctttctcgccacgttcgccggctttccccgtcaagctctaaatcgggggctccctttagggttccgatttagtgctttacggcacctcgaccccaaaaaacttgattagggtgatggttcacgtagtgggccatcgccctgatagacggtttttcgccctttgacgttggagtccacgttctttaatagtggactcttgttccaaactggaacaacactcaaccctatctcggtctattcttttgatttataagggattttgccgatttcggcctattggttaaaaaatgagctgatttaacaaaaatttaacgcgaattttaacaaaatattaacgcttacaatttcctgatgcggtattttctccttacgcatctgtgcggtatttcacaccgcatatcgaccggtcgaggagaacttctagtatatctacatacctaatattattgccttattaaaaatggaatcccaacaattacatcaaaatccacattctcttcaaaatcaattgtcctgtacttccttgttcatgtgtgttcaaaaacgttatatttataggataattatactctatttctcaacaagtaattggttgtttggccgagcggtctaaggcgcctgattcaagaaatatcttgaccgcagttaactgtgggaatactcaggtatcgtaagatgcaagagttcgaatctcttagcaaccattatttttttcctcaacataacgagaacacacaggggcgctatcgcacagaatcaaattcgatgactggaaattttttgttaatttcagaggtcgcctgacgcatatacctttttcaactgaaaaattgggagaaaaaggaaaggtgagagcgccggaaccggcttttcatatagaatagagaagcgttcatgactaaatgcttgcatcacaatacttgaagttgacaatattatttaaggacctattgttttttccaataggtggttagcaatcgtcttactttctaacttttcttaccttttacatttcagcaatatatatatatatatttcaaggatataccattctaatgtctgcccctaagaagatcgtcgttttgccaggtgaccacgttggtcaagaaatcacagccgaagccattaaggttcttaaagctatttctgatgttcgttccaatgtcaagttcgatttcgaaaatcatttaattggtggtgctgctatcgatgctacaggtgttccacttccagatgaggcgctggaagcctccaagaaggctgatgccgttttgttaggtgctgtgggtggtcctaaatggggtaccggtagtgttagacctgaacaaggtttactaaaaatccgtaaagaacttcaattgtacgccaacttaagaccatgtaactttgcatccgactctcttttagacttatctccaatcaagccacaatttgctaaaggtactgacttcgttgttgtcagagaattagtgggaggtatttactttggtaagagaaaggaagacgatggtgatggtgtcgcttgggatagtgaacaatacaccgttccagaagtgcaaagaatcacaagaatggccgctttcatggccctacaacatgagccaccattgcctatttggtccttggataaagctaatgttttggcctcttcaagattatggagaaaaactgtggaggaaaccatcaagaacgaattccctacattgaaggttcaacatcaattgattgattctgccgccatgatcctagttaagaacccaacccacctaaatggtattataatcaccagcaacatgtttggtgatatcatctccgatgaagcctccgttatcccaggttccttgggtttgttgccatctgcgtccttggcctctttgccagacaagaacaccgcatttggtttgtacgaaccatgccacggttctgctccagatttgccaaagaataaggtcaaccctatcgccactatcttgtctgctgcaatgatgttgaaattgtcattgaacttgcctgaagaaggtaaggccattgaagatgcagttaaaaaggttttggatgcaggtatcagaactggtgatttaggtggttccaacagtaccaccgaagtcggtgatgctgtcgccgaagaagttaagaaaatccttgcttaaaaagattctctttttttatgatatttgtacataaactttataaatgaaattcataatagaaacgacacgaaattacaaaatggaatatgttcatagggtagacgaaactatatacgcaatctacatacatttatcaagaaggagaaaaaggaggatgtaaaggaatacaggtaagcaaattgatactaatggctcaacgtgataaggaaaaagaattgcactttaacattaatattgacaaggaggagggcaccacacaaaaagttaggtgtaacagaaaatcatgaaactatgattcctaatttatatattggaggattttctctaaaaaaaaaaaaatacaacaaataaaaaacactcaatgacctgaccatttgatggagtttaagtcaataccttcttgaaccatttcccataatggtgaaagttccctcaagaattttactctgtcagaaacggccttaacgacgtagtcgatatggtgcactctcagtacaatctgctctgatgccgcatagttaagccagccccgacacccgccaacacccgctgacgcgccctgacgggcttgtctgctcccggcatccgcttacagacaagctgtgaccgtctccgggagctgcatgtgtcagaggttttcaccgtcatcaccgaaacgcgcgagacgaaagggcctcgtgatacgcctatttttataggttaatgtcatgataataatggtttcttagacggatcgcttgcctgtaacttacacgcgcctcgtatcttttaatgatggaataatttgggaatttactctgtgtttatttatttttatgttttgtatttggattttagaaagtaaataaagaaggtagaagagttacggaatgaagaaaaaaaaataaacaaaggtttaaaaaatttcaacaaaaagcgtactttacatatatatttattagacaagaaaagcagattaaatagatatacattcgattaacgataagtaaaatgtaaaatcacaggattttcgtgtgtggtcttctacacagacaagatgaaacaattcggcattaatacctgagagcaggaagagcaagataaaaggtagtatttgttggcgatccccctagagtcttttacatcttcggaaaacaaaaactattttttctttaatttctttttttactttctatttttaatttatatatttatattaaaaaatttaaattataattatttttatagcacgtgatgaaaaggacccaggtggcacttttcggggaaatgtgcgcggaacccctatttgtttatttttctaaatacattcaaatatgtatccgctcatgagacaataaccctgataaatgcttcaataatattgaaaaaggaagagtatgagtattcaacatttccgtgtcgcccttattcccttttttgcggcattttgccttcctgtttttgctcacccagaaacgctggtgaaagtaaaagatgctgaagatcagttgggtgcacgagtgggttacatcgaactggatctcaacagcggtaagatccttgagagttttcgccccgaagaacgttttccaatgatgagcacttttaaagttctgctatgtggcgcggtattatcccgtattgacgccgggcaagagcaactcggtcgccgcatacactattctcagaatgacttggttgagtactcaccagtcacagaaaagcatcttacggatggcatgacagtaagagaattatgcagtgctgccataaccatgagtgataacactgcggccaacttacttctgacaacgatcggaggaccgaaggagctaaccgcttttttgcacaacatgggggatcatgtaactcgccttgatcgttgggaaccggagctgaatgaagccataccaaacgacgagcgtgacaccacgatgcctgtagcaatggcaacaacgttgcgcaaactattaactggcgaactacttactctagcttcccggcaacaattaatagactggatggaggcggataaagttgcaggaccacttctgcgctcggcccttccggctggctggtttattgctgataaatctggagccggtgagcgtgggtctcgcggtatcattgcagcactggggccagatggtaagccctcccgtatcgtagttatctacacgacggggagtcaggcaactatggatgaacgaaatagacagatcgctgagataggtgcctcactgattaagcattggtaactgtcagaccaagtttactcatatatactttagattgatttaaaacttcatttttaatttaaaaggatctaggtgaagatcctttttgataatctcatgaccaaaatcccttaacgtgagttttcgttccactgagcgtcagaccccgtagaaaagatcaaaggatcttcttgagatcctttttttctgcgcgtaatctgctgcttgcaaacaaaaaaaccaccgctaccagcggtggtttgtttgccggatcaagagctaccaactctttttccgaaggtaactggcttcagcagagcgcagataccaaatactgttcttctagtgtagccgtagttaggccaccacttcaagaactctgtagcaccgcctacatacctcgctctgctaatcctgttaccagtggctgctgccagtggcgataagtcgtgtcttaccgggttggactcaagacgatagttaccggataaggcgcagcggtcgggctgaacggggggttcgtgcacacagcccagcttggagcgaacgacctacaccgaactgagatacctacagcgtgagctatgagaaagcgccacgcttcccgaagggagaaaggcggacaggtatccggtaagcggcagggtcggaacaggagagcgcacgagggagcttccagggggaaacgcctggtatctttatagtcctgtcgggtttcgccacctctgacttgagcgtcgatttttgtgatgctcgtcaggggggcggagcctatggaaaaacgccagcaacgcggcctttttacggttcctggccttttgctggccttttgctcacatgttctttcctgcgttatcccctgattctgtggataaccgtattaccgcctttgagtgagctgataccgctcgccgcagccgaacgaccgagcgcagcgagtcagtgagcgaggaagcggaagagcgcccaatacgcaaaccgcctctccccgcgcgttggccgattcattaatgcagctggcacgacaggtttcccgactggaaagcgggcagtgagcgcaacgcaattaatgtgagttagctcactcattaggcaccccaggctttacactttatgcttccggctcgtatgttgtgtggaattgtgagcggataacaatttcacacaggaaacagctatgaccatgattacgccaagctcgaaattaaccctcactaaagggaacaaaagctggtaccaattccttgaattttcaaaaattcttactttttttttggatggacgcaaagaagtttaataatcatattacatggcattaccaccatatacatatccatatctaatcttacttatatgttgtggaaatgtaaagagccccattatcttagcctaaaaaaaccttctctttggaactttcagtaatacgcttaactgctcattgctatattgaagta

SEQ ID NO: 7 - DNA, 6338 bp, synthetic construct
  misc_feature 1..6338: note = Plasmid PW27; note (original language) = Plásmido PW27
  source 1..6338: mol_type = other DNA
cggattagaagccgccgagcgggtgacagccctccgaaggaagactctcctccgtgcgtcctcgtcttcaccggtcgcgttcctgaaacgcagatgtgcctcgcgccgcactgctccgaacaataaagattctacaatactagcttttatggttatgaagaggaaaaattggcagtaacctggccccacaaaccttcaaatgaacgaatcaaattaacaaccataggatgataatgcgattagttttttagccttatttctggggtaattaatcagcgaagcgatgatttttgatctattaacagatatataaatgcaaaaactgcataaccactttaactaatactttcaacattttcggtttgtattacttcttattcaaatgtaataaaagtatcaacaaaaaattgttaatatacctctatactttaacgtcaaggagaaaaaaccccggatcgaattccctacttcatacattttcaattaagatgcagttacttcgctgtttttcaatattttctgttattgcttcagttttagcacaggaactgacaactatatgcgagcaaatcccctcaccaactttagaatcgacgccgtactctttgtcaacgactactattttggccaacgggaaggcaatgcaaggagtttttgaatattacaaatcagtaacgtttgtcagtaattgcggttctcacccctcaacaactagcaaaggcagccccataaacacacagtatgtttttaaggacaatagctcgacgattgaaggtagatacccatacgacgttccagactacgctctgcagttggttccaagaggttctctgcaggctagtggtggaggaggctctggtggaggcggtagcggaggcggagggtcggctagctgcggtggcggcggtactagcaaaatttctcattttttgaaaatggaatctttgaattttattagagctcatactccatatattaatatttacaattgtgaaccagctaatccatctgaaaaaaattctccatctactcaatattgttattctattcaatcttcccaggtcgactgcgggggcggatccgaacaaaagcttatttctgaagaggacttgtaatagctcgagatctgataacaacagtgtagatgtaacaaaatcgactttgttcccactgtacttttagctcgtacaaaatacaatatacttttcatttctccgtaaacaacatgttttcccatgtaatatccttttctatttttcgttccgttaccaactttacacatactttatatagctattcacttctatacactaaaaaactaagacaattttaattttgctgcctgccatatttcaatttgttataaattcctataatttatcctattagtagctaaaaaaagatgaatgtgaatcgaatcctaagagaattgagctccaattcgccctatagtgagtcgtattacaattcactggccgtcgttttacaacgtcgtgactgggaaaaccctggcgttacccaacttaatcgccttgcagcacatccccctttcgccagctggcgtaatagcgaagaggcccgcaccgatcgcctttcccaacagttgcgcagcctgaatggcgaatggacgcgccctgtagcggcgcattaagcgcggcgggtgtggtggttacgcgcagcgtgaccgctacacttgccagcgccctagcgcccgctcctttcgctttcttcccttcctttctcgccacgttcgccggctttccccgtcaagctctaaatcgggggctccctttagggttccgatttagtgctttacggcacctcgaccccaaaaaacttgattagggtgatggttcacgtagtgggccatcgccctgatagacggtttttcgccctttgacgttggagtccacgttctttaatagtggactcttgttccaaactggaacaacactcaaccctatctcggtctattcttttgatttataagggattttgccgatttcggcctattggttaaaaaatgagctgatttaacaaaaatttaacgcgaattttaacaaaatattaacgcttacaatttcctgatgcggtattttctccttacgcatctgtgcggtatttcacaccgcatagatcggcaagtgcacaaacaatacttaaataaatactactcagtaataacctatttcttagcatttttgacgaaatttgctattttgttagagtcttttacaccatttgtctccacacctccgcttacatcaacaccaataacgccatttaatctaagcgcatcaccaacattttctggcgtcagtccaccagctaacataaaatgtaagctttcggggctctcttgccttccaacccagtcagaaatcgagttccaatccaaaagttcacctgtcccacctgcttctgaatcaaacaagggaataaacgaatgaggtttctgtgaagctgcactgagtagtatgttgcagtcttttggaaatacgagtcttttaataactggcaaaccgaggaactcttggtattcttgccacgactcatctccatgcagttggacgatatcaatgccgtaatcattgaccagagccaaaacatcctccttaggttgattacgaaacacgccaaccaagtatttcggagtgcctgaactatttttatatgcttttacaagacttgaaattttccttgcaataaccgggtcaattgttctctttctattgggcacacatataatacccagcaagtcagcatcggaatctagagcacattctgcggcctctgtgctctgcaagccgcaaactttcaccaatggaccagaactacctgtgaaattaataacagacatactccaagctgcctttgtgtgcttaatcacgtatactcacgtgctcaatagtcaccaatgccctccctcttggccctctccttttcttttttcgaccgaattaattcttaatcggcaaaaaaagaaaagctccggatcaagattgtacgtaaggtgacaagctatttttcaataaagaatatcttccactactgccatctggcgtcataactgcaaagtacacatatattacgatgctgttctattaaatgcttcctatattatatatatagtaatgtcgtgatctatggtgcactctcagtacaatctgctctgatgccgcatagttaagccagccccgacacccgccaacacccgctgacgcgccctgacgggcttgtctgctcccggcatccgcttacagacaagctgtgaccgtctccgggagctgcatgtgtcagaggttttcaccgtcatcaccgaaacgcgcgagacgaaagggcctcgtgatacgcctatttttataggttaatgtcatgataataatggtttcttagacggatcgcttgcctgtaacttacacgcgcctcgtatcttttaatgatggaataatttgggaatttactctgtgtttatttatttttatgttttgtatttggattttagaaagtaaataaagaaggtagaagagttacggaatgaagaaaaaaaaataaacaaaggtttaaaaaatttcaacaaaaagcgtactttacatatatatttattagacaagaaaagcagattaaatagatatacattcgattaacgataagtaaaatgtaaaatcacaggattttcgtgtgtggtcttctacacagacaagatgaaacaattcggcattaatacctgagagcaggaagagcaagataaaaggtagtatttgttggcgatccccctagagtcttttacatcttcggaaaacaaaaactattttttctttaatttctttttttactttctatttttaatttatatatttatattaaaaaatttaaattataattatttttatagcacgtgatgaaaaggacccaggtggcacttttcggggaaatgtgcgcggaacccctatttgtttatttttctaaatacattcaaatatgtatccgctcatgagacaataaccctgataaatgcttcaataatattgaaaaaggaagagtatgagtattcaacatttccgtgtcgcccttattcccttttttgcggcattttgccttcctgtttttgctcacccagaaacgctggtgaaagtaaaagatgctgaagatcagttgggtgcacgagtgggttacatcgaactggatctcaacagcggtaagatccttgagagttttcgccccgaagaacgttttccaatgatgagcacttttaaagttctgctatgtggcgcggtattatcccgtattgacgccgggcaagagcaactcggtcgccgcatacactattctcagaatgacttggttgagtactcaccagtcacagaaaagcatcttacggatggcatgacagtaagagaattatgcagtgctgccataaccatgagtgataacactgcggccaacttacttctgacaacgatcggaggaccgaaggagctaaccgcttttttgcacaacatgggggatcatgtaactcgccttgatcgttgggaaccggagctgaatgaagccataccaaacgacgagcgtgacaccacgatgcctgtagcaatggcaacaacgttgcgcaaactattaactggcgaactacttactctagcttcccggcaacaattaatagactggatggaggcggataaagttgcaggaccacttctgcgctcggcccttccggctggctggtttattgctgataaatctggagccggtgagcgtgggtctcgcggtatcattgcagcactggggccagatggtaagccctcccgtatcgtagttatctacacgacggggagtcaggcaactatggatgaacgaaatagacagatcgctgagataggtgcctcactgattaagcattggtaactgtcagaccaagtttactcatatatactttagattgatttaaaacttcatttttaatttaaaaggatctaggtgaagatcctttttgataatctcatgaccaaaatcccttaacgtgagttttcgttccactgagcgtcagaccccgtagaaaagatcaaaggatcttcttgagatcctttttttctgcgcgtaatctgctgcttgcaaacaaaaaaaccaccgctaccagcggtggtttgtttgccggatcaagagctaccaactctttttccgaaggtaactggcttcagcagagcgcagataccaaatactgttcttctagtgtagccgtagttaggccaccacttcaagaactctgtagcaccgcctacatacctcgctctgctaatcctgttaccagtggctgctgccagtggcgataagtcgtgtcttaccgggttggactcaagacgatagttaccggataaggcgcagcggtcgggctgaacggggggttcgtgcacacagcccagcttggagcgaacgacctacaccgaactgagatacctacagcgtgagctatgagaaagcgccacgcttcccgaagggagaaaggcggacaggtatccggtaagcggcagggtcggaacaggagagcgcacgagggagcttccagggggaaacgcctggtatctttatagtcctgtcgggtttcgccacctctgacttgagcgtcgatttttgtgatgctcgtcaggggggcggagcctatggaaaaacgccagcaacgcggcctttttacggttcctggccttttgctggccttttgctcacatgttctttcctgcgttatcccctgattctgtggataaccgtattaccgcctttgagtgagctgataccgctcgccgcagccgaacgaccgagcgcagcgagtcagtgagcgaggaagcggaagagcgcccaatacgcaaaccgcctctccccgcgcgttggccgattcattaatgcagctggcacgacaggtttcccgactggaaagcgggcagtgagcgcaacgcaattaatgtgagttagctcactcattaggcaccccaggctttacactttatgcttccggctcgtatgttgtgtggaattgtgagcggataacaatttcacacaggaaacagctatgaccatgattacgccaagctcgaaattaaccctcactaaagggaacaaaagctggtaccaattccttgaattttcaaaaattcttactttttttttggatggacgcaaagaagtttaataatcatattacatggcattaccaccatatacatatccatatctaatcttacttatatgttgtggaaatgtaaagagccccattatcttagcctaaaaaaaccttctctttggaactttcagtaatacgcttaactgctcattgctatattgaagta

SEQ ID NO: 8 - DNA, 6512 bp, synthetic construct
  misc_feature 1..6512: note = Plasmid PW28; note (original language) = Plásmido PW28
  source 1..6512: mol_type = other DNA
cggattagaagccgccgagcgggtgacagccctccgaaggaagactctcctccgtgcgtcctcgtcttcaccggtcgcgttcctgaaacgcagatgtgcctcgcgccgcactgctccgaacaataaagattctacaatactagcttttatggttatgaagaggaaaaattggcagtaacctggccccacaaaccttcaaatgaacgaatcaaattaacaaccataggatgataatgcgattagttttttagccttatttctggggtaattaatcagcgaagcgatgatttttgatctattaacagatatataaatgcaaaaactgcataaccactttaactaatactttcaacattttcggtttgtattacttcttattcaaatgtaataaaagtatcaacaaaaaattgttaatatacctctatactttaacgtcaaggagaaaaaaccccggatcgaattccctacttcatacattttcaattaagatgcagttacttcgctgtttttcaatattttctgttattgcttcagttttagcacaggaactgacaactatatgcgagcaaatcccctcaccaactttagaatcgacgccgtactctttgtcaacgactactattttggccaacgggaaggcaatgcaaggagtttttgaatattacaaatcagtaacgtttgtcagtaattgcggttctcacccctcaacaactagcaaaggcagccccataaacacacagtatgtttttaaggacaatagctcgacgattgaaggtagatacccatacgacgttccagactacgctctgcagttggttccaagaggttctctgcaggctagtggtggaggaggctctggtggaggcggtagcggaggcggagggtcggctagctgcggtggcggcggtactagcaaaatttctcattttttgaaaatggaatctttgaattttattagagctcatactccatatattaatatttacaattgtgaaccagctaatccatctgaaaaaaattctccatctactcaatattgttattctattcaatcttcccaggtcgactgcgggggcggatccgaacaaaagcttatttctgaagaggacttgtaatagctcgagatctgataacaacagtgtagatgtaacaaaatcgactttgttcccactgtacttttagctcgtacaaaatacaatatacttttcatttctccgtaaacaacatgttttcccatgtaatatccttttctatttttcgttccgttaccaactttacacatactttatatagctattcacttctatacactaaaaaactaagacaattttaattttgctgcctgccatatttcaatttgttataaattcctataatttatcctattagtagctaaaaaaagatgaatgtgaatcgaatcctaagagaattgagctccaattcgccctatagtgagtcgtattacaattcactggccgtcgttttacaacgtcgtgactgggaaaaccctggcgttacccaacttaatcgccttgcagcacatccccctttcgccagctggcgtaatagcgaagaggcccgcaccgatcgcctttcccaacagttgcgcagcctgaatggcgaatggacgcgccctgtagcggcgcattaagcgcggcgggtgtggtggttacgcgcagcgtgaccgctacacttgccagcgccctagcgcccgctcctttcgctttcttcccttcctttctcgccacgttcgccggctttccccgtcaagctctaaatcgggggctccctttagggttccgatttagtgctttacggcacctcgaccccaaaaaacttgattagggtgatggttcacgtagtgggccatcgccctgatagacggtttttcgccctttgacgttggagtccacgttctttaatagtggactcttgttccaaactggaacaacactcaaccctatctcggtctattcttttgatttataagggattttgccgatttcggcctattggttaaaaaatgagctgatttaacaaaaatttaacgcgaattttaacaaaatattaacgtttacaatttcctgatgcggtattttctccttacgcatctgtgcggtatttcacaccgcatagatccgtcgagttcaagagaaaaaaaaagaaaaagcaaaaagaaaaaaggaaagcgcgcctcgttcagaatgacacgtatagaatgatgcattaccttgtcatcttcagtatcatactgttcgtatacatacttactgacattcataggtatacatatatacacatgtatatatatcgtatgctgcagctttaaataatcggtgtcactacataagaacacctttggtggagggaacatcgttggtaccattgggcgaggtggcttctcttatggcaaccgcaagagccttgaacgcactctcactacggtgatgatcattcttgcctcgcagacaatcaacgtggagggtaattctgctagcctctgcaaagctttcaagaaaatgcgggatcatctcgcaagagagatctcctactttctccctttgcaaaccaagttcgacaactgcgtacggcctgttcgaaagatctaccaccgctctggaaagtgcctcatccaaaggcgcaaatcctgatccaaacctttttactccacgcgccagtagggcctctttaaaagcttgaccgagagcaatcccgcagtcttcagtggtgtgatggtcgtctatgtgtaagtcaccaatgcactcaacgattagcgaccagccggaatgcttggccagagcatgtatcatatggtccagaaaccctatacctgtgtggacgttaatcacttgcgattgtgtggcctgttctgctactgcttctgcctctttttctgggaagatcgagtgctctatcgctaggggaccaccctttaaagagatcgcaatctgaatcttggtttcatttgtaatacgctttactagggctttctgctctgtcatctttgccttcgtttatcttgcctgctcattttttagtatattcttcgaagaaatcacattactttatataatgtataattcattatgtgataatgccaatcgctaagaaaaaaaaagagtcatccgctaggggaaaaaaaaaaatgaaaatcattaccgaggcataaaaaaatatagagtgtactagaggaggccaagagtaatagaaaaagaaaattgcgggaaaggactgtgttatgacttccctgactaatgccgtgttcaaacgatacctggcagtgactcctagcgctcaccaagctcttaaaacgggaatttatggtgcactctcagtacaatctgctctgatgccgcatagttaagccagccccgacacccgccaacacccgctgacgcgccctgacgggcttgtctgctcccggcatccgcttacagacaagctgtgaccgtctccgggagctgcatgtgtcagaggttttcaccgtcatcaccgaaacgcgcgagacgaaagggcctcgtgatacgcctatttttataggttaatgtcatgataataatggtttcttagacggatcgcttgcctgtaacttacacgcgcctcgtatcttttaatgatggaataatttgggaatttactctgtgtttatttatttttatgttttgtatttggattttagaaagtaaataaagaaggtagaagagttacggaatgaagaaaaaaaaataaacaaaggtttaaaaaatttcaacaaaaagcgtactttacatatatatttattagacaagaaaagcagattaaatagatatacattcgattaacgataagtaaaatgtaaaatcacaggattttcgtgtgtggtcttctacacagacaagatgaaacaattcggcattaatacctgagagcaggaagagcaagataaaaggtagtatttgttggcgatccccctagagtcttttacatcttcggaaaacaaaaactattttttctttaatttctttttttactttctatttttaatttatatatttatattaaaaaatttaaattataattatttttatagcacgtgatgaaaaggacccaggtggcacttttcggggaaatgtgcgcggaacccctatttgtttatttttctaaatacattcaaatatgtatccgctcatgagacaataaccctgataaatgcttcaataatattgaaaaaggaagagtatgagtattcaacatttccgtgtcgcccttattcccttttttgcggcattttgccttcctgtttttgctcacccagaaacgctggtgaaagtaaaagatgctgaagatcagttgggtgcacgagtgggttacatcgaactggatctcaacagcggtaagatccttgagagttttcgccccgaagaacgttttccaatgatgagcacttttaaagttctgctatgtggcgcggtattatcccgtattgacgccgggcaagagcaactcggtcgccgcatacactattctcagaatgacttggttgagtactcaccagtcacagaaaagcatcttacggatggcatgacagtaagagaattatgcagtgctgccataaccatgagtgataacactgcggccaacttacttctgacaacgatcggaggaccgaaggagctaaccgcttttttgcacaacatgggggatcatgtaactcgccttgatcgttgggaaccggagctgaatgaagccataccaaacgacgagcgtgacaccacgatgcctgtagcaatggcaacaacgttgcgcaaactattaactggcgaactacttactctagcttcccggcaacaattaatagactggatggaggcggataaagttgcaggaccacttctgcgctcggcccttccggctggctggtttattgctgataaatctggagccggtgagcgtgggtctcgcggtatcattgcagcactggggccagatggtaagccctcccgtatcgtagttatctacacgacggggagtcaggcaactatggatgaacgaaatagacagatcgctgagataggtgcctcactgattaagcattggtaactgtcagaccaagtttactcatatatactttagattgatttaaaacttcatttttaatttaaaaggatctaggtgaagatcctttttgataatctcatgaccaaaatcccttaacgtgagttttcgttccactgagcgtcagaccccgtagaaaagatcaaaggatcttcttgagatcctttttttctgcgcgtaatctgctgcttgcaaacaaaaaaaccaccgctaccagcggtggtttgtttgccggatcaagagctaccaactctttttccgaaggtaactggcttcagcagagcgcagataccaaatactgttcttctagtgtagccgtagttaggccaccacttcaagaactctgtagcaccgcctacatacctcgctctgctaatcctgttaccagtggctgctgccagtggcgataagtcgtgtcttaccgggttggactcaagacgatagttaccggataaggcgcagcggtcgggctgaacggggggttcgtgcacacagcccagcttggagcgaacgacctacaccgaactgagatacctacagcgtgagctatgagaaagcgccacgcttcccgaagggagaaaggcggacaggtatccggtaagcggcagggtcggaacaggagagcgcacgagggagcttccagggggaaacgcctggtatctttatagtcctgtcgggtttcgccacctctgacttgagcgtcgatttttgtgatgctcgtcaggggggcggagcctatggaaaaacgccagcaacgcggcctttttacggttcctggccttttgctggccttttgctcacatgttctttcctgcgttatcccctgattctgtggataaccgtattaccgcctttgagtgagctgataccgctcgccgcagccgaacgaccgagcgcagcgagtcagtgagcgaggaagcggaagagcgcccaatacgcaaaccgcctctccccgcgcgttggccgattcattaatgcagctggcacgacaggtttcccgactggaaagcgggcagtgagcgcaacgcaattaatgtgagttagctcactcattaggcaccccaggctttacactttatgcttccggctcgtatgttgtgtggaattgtgagcggataacaatttcacacaggaaacagctatgaccatgattacgccaagctcgaaattaaccctcactaaagggaacaaaagctggtaccaattccttgaattttcaaaaattcttactttttttttggatggacgcaaagaagtttaataatcatattacatggcattaccaccatatacatatccatatctaatcttacttatatgttgtggaaatgtaaagagccccattatcttagcctaaaaaaaccttctctttggaactttcagtaatacgcttaactgctcattgctatattgaagta

SEQ ID NO: 9 - DNA, 7556 bp, synthetic construct
  misc_feature 1..7556: note = Plasmid PW29; note (original language) = Plásmido PW29
  source 1..7556: mol_type = other DNA
cggattagaagccgccgagcgggtgacagccctccgaaggaagactctcctccgtgcgtcctcgtcttcaccggtcgcgttcctgaaacgcagatgtgcctcgcgccgcactgctccgaacaataaagattctacaatactagcttttatggttatgaagaggaaaaattggcagtaacctggccccacaaaccttcaaatgaacgaatcaaattaacaaccataggatgataatgcgattagttttttagccttatttctggggtaattaatcagcgaagcgatgatttttgatctattaacagatatataaatgcaaaaactgcataaccactttaactaatactttcaacattttcggtttgtattacttcttattcaaatgtaataaaagtatcaacaaaaaattgttaatatacctctatactttaacgtcaaggagaaaaaaccccggatcgaattccctacttcatacattttcaattaagatgcagttacttcgctgtttttcaatattttctgttattgcttcagttttagcacaggaactgacaactatatgcgagcaaatcccctcaccaactttagaatcgacgccgtactctttgtcaacgactactattttggccaacgggaaggcaatgcaaggagtttttgaatattacaaatcagtaacgtttgtcagtaattgcggttctcacccctcaacaactagcaaaggcagccccataaacacacagtatgtttttaaggacaatagctcgacgattgaaggtagatacccatacgacgttccagactacgctctgcagttggttccaagaggttctctgcaggctagtggtggaggaggctctggtggaggcggtagcggaggcggagggtcggctagctgcggtggcggcggtactagcaaaatttctcattttttgaaaatggaatctttgaattttattagagctcatactccatatattaatatttacaattgtgaaccagctaatccatctgaaaaaaattctccatctactcaatattgttattctattcaatcttcccaggtcgactgcgggggcggatccgaacaaaagcttatttctgaagaggacttgtaatagctcgagatctgataacaacagtgtagatgtaacaaaatcgactttgttcccactgtacttttagctcgtacaaaatacaatatacttttcatttctccgtaaacaacatgttttcccatgtaatatccttttctatttttcgttccgttaccaactttacacatactttatatagctattcacttctatacactaaaaaactaagacaattttaattttgctgcctgccatatttcaatttgttataaattcctataatttatcctattagtagctaaaaaaagatgaatgtgaatcgaatcctaagagaattgagctccaattcgccctatagtgagtcgtattacaattcactggccgtcgttttacaacgtcgtgactgggaaaaccctggcgttacccaacttaatcgccttgcagcacatccccctttcgccagctggcgtaatagcgaagaggcccgcaccgatcgcctttcccaacagttgcgcagcctgaatggcgaatggacgcgccctgtagcggcgcattaagcgcggcgggtgtggtggttacgcgcagcgtgaccgctacacttgccagcgccctagcgcccgctcctttcgctttcttcccttcctttctcgccacgttcgccggctttccccgtcaagctctaaatcgggggctccctttagggttccgatttagtgctttacggcacctcgaccccaaaaaacttgattagggtgatggttcacgtagtgggccatcgccctgatagacggtttttcgccctttgacgttggagtccacgttctttaatagtggactcttgttccaaactggaacaacactcaaccctatctcggtctattcttttgatttataagggattttgccgatttcggcctattggttaaaaaatgagctgatttaacaaaaatttaacgcgaattttaacaaaatattaacgcttacaatttcctgatgcggtattttctccttacgcatctgtgcggtatttcacaccgcatatcgaccggtcgaggagaacttctagtatatctacatacctaatattattgccttattaaaaatggaatcccaacaattacatcaaaatccacattctcttcaaaatcaattgtcctgtacttccttgttcatgtgtgttcaaaaacgttatatttataggataattatactctatttctcaacaagtaattggttgtttggccgagcggtctaaggcgcctgattcaagaaatatcttgaccgcagttaactgtgggaatactcaggtatcgtaagatgcaagagttcgaatctcttagcaaccattatttttttcctcaacataacgagaacacacaggggcgctatcgcacagaatcaaattcgatgactggaaattttttgttaatttcagaggtcgcctgacgcatatacctttttcaactgaaaaattgggagaaaaaggaaaggtgagagcgccggaaccggcttttcatatagaatagagaagcgttcatgactaaatgcttgcatcacaatacttgaagttgacaatattatttaaggacctattgttttttccaataggtggttagcaatcgtcttactttctaacttttcttaccttttacatttcagcaatatatatatatatatttcaaggatataccattctaatgtctgcccctaagaagatcgtcgttttgccaggtgaccacgttggtcaagaaatcacagccgaagccattaaggttcttaaagctatttctgatgttcgttccaatgtcaagttcgatttcgaaaatcatttaattggtggtgctgctatcgatgctacaggtgttccacttccagatgaggcgctggaagcctccaagaaggctgatgccgttttgttaggtgctgtgggtggtcctaaatggggtaccggtagtgttagacctgaacaaggtttactaaaaatccgtaaagaacttcaattgtacgccaacttaagaccatgtaactttgcatccgactctcttttagacttatctccaatcaagccacaatttgctaaaggtactgacttcgttgttgtcagagaattagtgggaggtatttactttggtaagagaaaggaagacgatggtgatggtgtcgcttgggatagtgaacaatacaccgttccagaagtgcaaagaatcacaagaatggccgctttcatggccctacaacatgagccaccattgcctatttggtccttggataaagctaatgttttggcctcttcaagattatggagaaaaactgtggaggaaaccatcaagaacgaattccctacattgaaggttcaacatcaattgattgattctgccgccatgatcctagttaagaacccaacccacctaaatggtattataatcaccagcaacatgtttggtgatatcatctccgatgaagcctccgttatcccaggttccttgggtttgttgccatctgcgtccttggcctctttgccagacaagaacaccgcatttggtttgtacgaaccatgccacggttctgctccagatttgccaaagaataaggtcaaccctatcgccactatcttgtctgctgcaatgatgttgaaattgtcattgaacttgcctgaagaaggtaaggccattgaagatgcagttaaaaaggttttggatgcaggtatcagaactggtgatttaggtggttccaacagtaccaccgaagtcggtgatgctgtcgccgaagaagttaagaaaatccttgcttaaaaagattctctttttttatgatatttgtacataaactttataaatgaaattcataatagaaacgacacgaaattacaaaatggaatatgttcatagggtagacgaaactatatacgcaatctacatacatttatcaagaaggagaaaaaggaggatgtaaaggaatacaggtaagcaaattgatactaatggctcaacgtgataaggaaaaagaattgcactttaacattaatattgacaaggaggagggcaccacacaaaaagttaggtgtaacagaaaatcatgaaactatgattcctaatttatatattggaggattttctctaaaaaaaaaaaaatacaacaaataaaaaacactcaatgacctgaccatttgatggagtttaagtcaataccttcttgaaccatttcccataatggtgaaagttccctcaagaattttactctgtcagaaacggccttaacgacgtagtcgatatggtgcactctcagtacaatctgctctgatgccgcatagttaagccagccccgacacccgccaacacccgctgacgcgccctgacgggcttgtctgctcccggcatccgcttacagacaagctgtgaccgtctccgggagctgcatgtgtcagaggttttcaccgtcatcaccgaaacgcgcgagacgaaagggcctcgtgatacgcctatttttataggttaatgtcatgataataatggtttcttagacggatcgcttgcctgtaacttacacgcgcctcgtatcttttaatgatggaataatttgggaatttactctgtgtttatttatttttatgttttgtatttggattttagaaagtaaataaagaaggtagaagagttacggaatgaagaaaaaaaaataaacaaaggtttaaaaaatttcaacaaaaagcgtactttacatatatatttattagacaagaaaagcagattaaatagatatacattcgattaacgataagtaaaatgtaaaatcacaggattttcgtgtgtggtcttctacacagacaagatgaaacaattcggcattaatacctgagagcaggaagagcaagataaaaggtagtatttgttggcgatccccctagagtcttttacatcttcggaaaacaaaaactattttttctttaatttctttttttactttctatttttaatttatatatttatattaaaaaatttaaattataattatttttatagcacgtgatgaaaaggacccaggtggcacttttcggggaaatgtgcgcggaacccctatttgtttatttttctaaatacattcaaatatgtatccgctcatgagacaataaccctgataaatgcttcaataatattgaaaaaggaagagtatgagtattcaacatttccgtgtcgcccttattcccttttttgcggcattttgccttcctgtttttgctcacccagaaacgctggtgaaagtaaaagatgctgaagatcagttgggtgcacgagtgggttacatcgaactggatctcaacagcggtaagatccttgagagttttcgccccgaagaacgttttccaatgatgagcacttttaaagttctgctatgtggcgcggtattatcccgtattgacgccgggcaagagcaactcggtcgccgcatacactattctcagaatgacttggttgagtactcaccagtcacagaaaagcatcttacggatggcatgacagtaagagaattatgcagtgctgccataaccatgagtgataacactgcggccaacttacttctgacaacgatcggaggaccgaaggagctaaccgcttttttgcacaacatgggggatcatgtaactcgccttgatcgttgggaaccggagctgaatgaagccataccaaacgacgagcgtgacaccacgatgcctgtagcaatggcaacaacgttgcgcaaactattaactggcgaactacttactctagcttcccggcaacaattaatagactggatggaggcggataaagttgcaggaccacttctgcgctcggcccttccggctggctggtttattgctgataaatctggagccggtgagcgtgggtctcgcggtatcattgcagcactggggccagatggtaagccctcccgtatcgtagttatctacacgacggggagtcaggcaactatggatgaacgaaatagacagatcgctgagataggtgcctcactgattaagcattggtaactgtcagaccaagtttactcatatatactttagattgatttaaaacttcatttttaatttaaaaggatctaggtgaagatcctttttgataatctcatgaccaaaatcccttaacgtgagttttcgttccactgagcgtcagaccccgtagaaaagatcaaaggatcttcttgagatcctttttttctgcgcgtaatctgctgcttgcaaacaaaaaaaccaccgctaccagcggtggtttgtttgccggatcaagagctaccaactctttttccgaaggtaactggcttcagcagagcgcagataccaaatactgttcttctagtgtagccgtagttaggccaccacttcaagaactctgtagcaccgcctacatacctcgctctgctaatcctgttaccagtggctgctgccagtggcgataagtcgtgtcttaccgggttggactcaagacgatagttaccggataaggcgcagcggtcgggctgaacggggggttcgtgcacacagcccagcttggagcgaacgacctacaccgaactgagatacctacagcgtgagctatgagaaagcgccacgcttcccgaagggagaaaggcggacaggtatccggtaagcggcagggtcggaacaggagagcgcacgagggagcttccagggggaaacgcctggtatctttatagtcctgtcgggtttcgccacctctgacttgagcgtcgatttttgtgatgctcgtcaggggggcggagcctatggaaaaacgccagcaacgcggcctttttacggttcctggccttttgctggccttttgctcacatgttctttcctgcgttatcccctgattctgtggataaccgtattaccgcctttgagtgagctgataccgctcgccgcagccgaacgaccgagcgcagcgagtcagtgagcgaggaagcggaagagcgcccaatacgcaaaccgcctctccccgcgcgttggccgattcattaatgcagctggcacgacaggtttcccgactggaaagcgggcagtgagcgcaacgcaattaatgtgagttagctcactcattaggcaccccaggctttacactttatgcttccggctcgtatgttgtgtggaattgtgagcggataacaatttcacacaggaaacagctatgaccatgattacgccaagctcgaaattaaccctcactaaagggaacaaaagctggtaccaattccttgaattttcaaaaattcttactttttttttggatggacgcaaagaagtttaataatcatattacatggcattaccaccatatacatatccatatctaatcttacttatatgttgtggaaatgtaaagagccccattatcttagcctaaaaaaaccttctctttggaactttcagtaatacgcttaactgctcattgctatattgaagta

SEQ ID NO: 10 - DNA, 6329 bp, synthetic construct
  misc_feature 1..6329: note = Plasmid PW30; note (original language) = Plásmido PW30
  source 1..6329: mol_type = other DNA
cggattagaagccgccgagcgggtgacagccctccgaaggaagactctcctccgtgcgtcctcgtcttcaccggtcgcgttcctgaaacgcagatgtgcctcgcgccgcactgctccgaacaataaagattctacaatactagcttttatggttatgaagaggaaaaattggcagtaacctggccccacaaaccttcaaatgaacgaatcaaattaacaaccataggatgataatgcgattagttttttagccttatttctggggtaattaatcagcgaagcgatgatttttgatctattaacagatatataaatgcaaaaactgcataaccactttaactaatactttcaacattttcggtttgtattacttcttattcaaatgtaataaaagtatcaacaaaaaattgttaatatacctctatactttaacgtcaaggagaaaaaaccccggatcgaattccctacttcatacattttcaattaagatgcagttacttcgctgtttttcaatattttctgttattgcttcagttttagcacaggaactgacaactatatgcgagcaaatcccctcaccaactttagaatcgacgccgtactctttgtcaacgactactattttggccaacgggaaggcaatgcaaggagtttttgaatattacaaatcagtaacgtttgtcagtaattgcggttctcacccctcaacaactagcaaaggcagccccataaacacacagtatgtttttaaggacaatagctcgacgattgaaggtagatacccatacgacgttccagactacgctctgcaggctagtggtggaggaggctctggtggaggcggtagcggaggcggagggtcggctagctgcggtggcggcggtactagcaaaatttctcattttttgaaaatggaatctttgaattttattagagctcatactccatatattaatatttacaattgtgaaccagctaatccatctgaaaaaaattctccatctactcaatattgttattctattcaatcttcccaggtcgactgcgggggcggatccgaacaaaagcttatttctgaagaggacttgcaccaccaccaccaccactgactcgagatctgataacaacagtgtagatgtaacaaaatcgactttgttcccactgtacttttagctcgtacaaaatacaatatacttttcatttctccgtaaacaacatgttttcccatgtaatatccttttctatttttcgttccgttaccaactttacacatactttatatagctattcacttctatacactaaaaaactaagacaattttaattttgctgcctgccatatttcaatttgttataaattcctataatttatcctattagtagctaaaaaaagatgaatgtgaatcgaatcctaagagaattgagctccaattcgccctatagtgagtcgtattacaattcactggccgtcgttttacaacgtcgtgactgggaaaaccctggcgttacccaacttaatcgccttgcagcacatccccctttcgccagctggcgtaatagcgaagaggcccgcaccgatcgcctttcccaacagttgcgcagcctgaatggcgaatggacgcgccctgtagcggcgcattaagcgcggcgggtgtggtggttacgcgcagcgtgaccgctacacttgccagcgccctagcgcccgctcctttcgctttcttcccttcctttctcgccacgttcgccggctttccccgtcaagctctaaatcgggggctccctttagggttccgatttagtgctttacggcacctcgaccccaaaaaacttgattagggtgatggttcacgtagtgggccatcgccctgatagacggtttttcgccctttgacgttggagtccacgttctttaatagtggactcttgttccaaactggaacaacactcaaccctatctcggtctattcttttgatttataagggattttgccgatttcggcctattggttaaaaaatgagctgatttaacaaaaatttaacgcgaattttaacaaaatattaacgcttacaatttcctgatgcggtattttctccttacgcatctgtgcggtatttcacaccgcatagatcggcaagtgcacaaacaatacttaaataaatactactcagtaataacctatttcttagcatttttgacgaaatttgctattttgttagagtcttttacaccatttgtctccacacctccgcttacatcaacaccaataacgccatttaatctaagcgcatcaccaacattttctggcgtcagtccaccagctaacataaaatgtaagctttcggggctctcttgccttccaacccagtcagaaatcgagttccaatccaaaagttcacctgtcccacctgcttctgaatcaaacaagggaataaacgaatgaggtttctgtgaagctgcactgagtagtatgttgcagtcttttggaaatacgagtcttttaataactggcaaaccgaggaactcttggtattcttgccacgactcatctccatgcagttggacgatatcaatgccgtaatcattgaccagagccaaaacatcctccttaggttgattacgaaacacgccaaccaagtatttcggagtgcctgaactatttttatatgcttttacaagacttgaaattttccttgcaataaccgggtcaattgttctctttctattgggcacacatataatacccagcaagtcagcatcggaatctagagcacattctgcggcctctgtgctctgcaagccgcaaactttcaccaatggaccagaactacctgtgaaattaataacagacatactccaagctgcctttgtgtgcttaatcacgtatactcacgtgctcaatagtcaccaatgccctccctcttggccctctccttttcttttttcgaccgaattaattcttaatcggcaaaaaaagaaaagctccggatcaagattgtacgtaaggtgacaagctatttttcaataaagaatatcttccactactgccatctggcgtcataactgcaaagtacacatatattacgatgctgttctattaaatgcttcctatattatatatatagtaatgtcgtgatctatggtgcactctcagtacaatctgctctgatgccgcatagttaagccagccccgacacccgccaacacccgctgacgcgccctgacgggcttgtctgctcccggcatccgcttacagacaagctgtgaccgtctccgggagctgcatgtgtcagaggttttcaccgtcatcaccgaaacgcgcgagacgaaagggcctcgtgatacgcctatttttataggttaatgtcatgataataatggtttcttagacggatcgcttgcctgtaacttacacgcgcctcgtatcttttaatgatggaataatttgggaatttactctgtgtttatttatttttatgttttgtatttggattttagaaagtaaataaagaaggtagaagagttacggaatgaagaaaaaaaaataaacaaaggtttaaaaaatttcaacaaaaagcgtactttacatatatatttattagacaagaaaagcagattaaatagatatacattcgattaacgataagtaaaatgtaaaatcacaggattttcgtgtgtggtcttctacacagacaagatgaaacaattcggcattaatacctgagagcaggaagagcaagataaaaggtagtatttgttggcgatccccctagagtcttttacatcttcggaaaacaaaaactattttttctttaatttctttttttactttctatttttaatttatatatttatattaaaaaatttaaattataattatttttatagcacgtgatgaaaaggacccaggtggcacttttcggggaaatgtgcgcggaacccctatttgtttatttttctaaatacattcaaatatgtatccgctcatgagacaataaccctgataaatgcttcaataatattgaaaaaggaagagtatgagtattcaacatttccgtgtcgcccttattcccttttttgcggcattttgccttcctgtttttgctcacccagaaacgctggtgaaagtaaaagatgctgaagatcagttgggtgcacgagtgggttacatcgaactggatctcaacagcggtaagatccttgagagttttcgccccgaagaacgttttccaatgatgagcacttttaaagttctgctatgtggcgcggtattatcccgtattgacgccgggcaagagcaactcggtcgccgcatacactattctcagaatgacttggttgagtactcaccagtcacagaaaagcatcttacggatggcatgacagtaagagaattatgcagtgctgccataaccatgagtgataacactgcggccaacttacttctgacaacgatcggaggaccgaaggagctaaccgcttttttgcacaacatgggggatcatgtaactcgccttgatcgttgggaaccggagctgaatgaagccataccaaacgacgagcgtgacaccacgatgcctgtagcaatggcaacaacgttgcgcaaactattaactggcgaactacttactctagcttcccggcaacaattaatagactggatggaggcggataaagttgcaggaccacttctgcgctcggcccttccggctggctggtttattgctgataaatctggagccggtgagcgtgggtctcgcggtatcattgcagcactggggccagatggtaagccctcccgtatcgtagttatctacacgacggggagtcaggcaactatggatgaacgaaatagacagatcgctgagataggtgcctcactgattaagcattggtaactgtcagaccaagtttactcatatatactttagattgatttaaaacttcatttttaatttaaaaggatctaggtgaagatcctttttgataatctcatgaccaaaatcccttaacgtgagttttcgttccactgagcgtcagaccccgtagaaaagatcaaaggatcttcttgagatcctttttttctgcgcgtaatctgctgcttgcaaacaaaaaaaccaccgctaccagcggtggtttgtttgccggatcaagagctaccaactctttttccgaaggtaactggcttcagcagagcgcagataccaaatactgttcttctagtgtagccgtagttaggccaccacttcaagaactctgtagcaccgcctacatacctcgctctgctaatcctgttaccagtggctgctgccagtggcgataagtcgtgtcttaccgggttggactcaagacgatagttaccggataaggcgcagcggtcgggctgaacggggggttcgtgcacacagcccagcttggagcgaacgacctacaccgaactgagatacctacagcgtgagctatgagaaagcgccacgcttcccgaagggagaaaggcggacaggtatccggtaagcggcagggtcggaacaggagagcgcacgagggagcttccagggggaaacgcctggtatctttatagtcctgtcgggtttcgccacctctgacttgagcgtcgatttttgtgatgctcgtcaggggggcggagcctatggaaaaacgccagcaacgcggcctttttacggttcctggccttttgctggccttttgctcacatgttctttcctgcgttatcccctgattctgtggataaccgtattaccgcctttgagtgagctgataccgctcgccgcagccgaacgaccgagcgcagcgagtcagtgagcgaggaagcggaagagcgcccaatacgcaaaccgcctctccccgcgcgttggccgattcattaatgcagctggcacgacaggtttcccgactggaaagcgggcagtgagcgcaacgcaattaatgtgagttagctcactcattaggcaccccaggctttacactttatgcttccggctcgtatgttgtgtggaattgtgagcggataacaatttcacacaggaaacagctatgaccatgattacgccaagctcgaaattaaccctcactaaagggaacaaaagctggtaccaattccttgaattttcaaaaattcttactttttttttggatggacgcaaagaagtttaataatcatattacatggcattaccaccatatacatatccatatctaatcttacttatatgttgtggaaatgtaaagagccccattatcttagcctaaaaaaaccttctctttggaactttcagtaatacgcttaactgctcattgctatattgaagta

SEQ ID NO: 11 - DNA, 6503 bp, synthetic construct
  misc_feature 1..6503: note = Plasmid PW31; note (original language) = Plásmido PW31
  source 1..6503: mol_type = other DNA
cggattagaagccgccgagcgggtgacagccctccgaaggaagactctcctccgtgcgtcctcgtcttcaccggtcgcgttcctgaaacgcagatgtgcctcgcgccgcactgctccgaacaataaagattctacaatactagcttttatggttatgaagaggaaaaattggcagtaacctggccccacaaaccttcaaatgaacgaatcaaattaacaaccataggatgataatgcgattagttttttagccttatttctggggtaattaatcagcgaagcgatgatttttgatctattaacagatatataaatgcaaaaactgcataaccactttaactaatactttcaacattttcggtttgtattacttcttattcaaatgtaataaaagtatcaacaaaaaattgttaatatacctctatactttaacgtcaaggagaaaaaaccccggatcgaattccctacttcatacattttcaattaagatgcagttacttcgctgtttttcaatattttctgttattgcttcagttttagcacaggaactgacaactatatgcgagcaaatcccctcaccaactttagaatcgacgccgtactctttgtcaacgactactattttggccaacgggaaggcaatgcaaggagtttttgaatattacaaatcagtaacgtttgtcagtaattgcggttctcacccctcaacaactagcaaaggcagccccataaacacacagtatgtttttaaggacaatagctcgacgattgaaggtagatacccatacgacgttccagactacgctctgcaggctagtggtggaggaggctctggtggaggcggtagcggaggcggagggtcggctagctgcggtggcggcggtactagcaaaatttctcattttttgaaaatggaatctttgaattttattagagctcatactccatatattaatatttacaattgtgaaccagctaatccatctgaaaaaaattctccatctactcaatattgttattctattcaatcttcccaggtcgactgcgggggcggatccgaacaaaagcttatttctgaagaggacttgcaccaccaccaccaccactgactcgagatctgataacaacagtgtagatgtaacaaaatcgactttgttcccactgtacttttagctcgtacaaaatacaatatacttttcatttctccgtaaacaacatgttttcccatgtaatatccttttctatttttcgttccgttaccaactttacacatactttatatagctattcacttctatacactaaaaaactaagacaattttaattttgctgcctgccatatttcaatttgttataaattcctataatttatcctattagtagctaaaaaaagatgaatgtgaatcgaatcctaagagaattgagctccaattcgccctatagtgagtcgtattacaattcactggccgtcgttttacaacgtcgtgactgggaaaaccctggcgttacccaacttaatcgccttgcagcacatccccctttcgccagctggcgtaatagcgaagaggcccgcaccgatcgcctttcccaacagttgcgcagcctgaatggcgaatggacgcgccctgtagcggcgcattaagcgcggcgggtgtggtggttacgcgcagcgtgaccgctacacttgccagcgccctagcgcccgctcctttcgctttcttcccttcctttctcgccacgttcgccggctttccccgtcaagctctaaatcgggggctccctttagggttccgatttagtgctttacggcacctcgaccccaaaaaacttgattagggtgatggttcacgtagtgggccatcgccctgatagacggtttttcgccctttgacgttggagtccacgttctttaatagtggactcttgttccaaactggaacaacactcaaccctatctcggtctattcttttgatttataagggattttgccgatttcggcctattggttaaaaaatgagctgatttaacaaaaatttaacgcgaattttaacaaaatattaacgtttacaatttcctgatgcggtattttctccttacgcatctgtgcggtatttcacaccgcatagatccgtcgagttcaagagaaaaaaaaagaaaaagcaaaaagaaaaaaggaaagcgcgcctcgttcagaatgacacgtatagaatgatgcattaccttgtcatcttcagtatcatactgttcgtatacatacttactgacattcataggtatacatatatacacatgtatatatatcgtatgctgcagctttaaataatcggtgtcactacataagaacacctttggtggagggaacatcgttggtaccattgggcgaggtggcttctcttatggcaaccgcaagagccttgaacgcactctcactacggtgatgatcattcttgcctcgcagacaatcaacgtggagggtaattctgctagcctctgcaaagctttcaagaaaatgcgggatcatctcgcaagagagatctcctactttctccctttgcaaaccaagttcgacaactgcgtacggcctgttcgaaagatctaccaccgctctggaaagtgcctcatccaaaggcgcaaatcctgatccaaacctttttactccacgcgccagtagggcctctttaaaagcttgaccgagagcaatcccgcagtcttcagtggtgtgatggtcgtctatgtgtaagtcaccaatgcactcaacgattagcgaccagccggaatgcttggccagagcatgtatcatatggtccagaaaccctatacctgtgtggacgttaatcacttgcgattgtgtggcctgttctgctactgcttctgcctctttttctgggaagatcgagtgctctatcgctaggggaccaccctttaaagagatcgcaatctgaatcttggtttcatttgtaatacgctttactagggctttctgctctgtcatctttgccttcgtttatcttgcctgctcattttttagtatattcttcgaagaaatcacattactttatataatgtataattcattatgtgataatgccaatcgctaagaaaaaaaaagagtcatccgctaggggaaaaaaaaaaatgaaaatcattaccgaggcataaaaaaatatagagtgtactagaggaggccaagagtaatagaaaaagaaaattgcgggaaaggactgtgttatgacttccctgactaatgccgtgttcaaacgatacctggcagtgactcctagcgctcaccaagctcttaaaacgggaatttatggtgcactctcagtacaatctgctctgatgccgcatagttaagccagccccgacacccgccaacacccgctgacgcgccctgacgggcttgtctgctcccggcatccgcttacagacaagctgtgaccgtctccgggagctgcatgtgtcagaggttttcaccgtcatcaccgaaacgcgcgagacgaaagggcctcgtgatacgcctatttttataggttaatgtcatgataataatggtttcttagacggatcgcttgcctgtaacttacacgcgcctcgtatcttttaatgatggaataatttgggaatttactctgtgtttatttatttttatgttttgtatttggattttagaaagtaaataaagaaggtagaagagttacggaatgaagaaaaaaaaataaacaaaggtttaaaaaatttcaacaaaaagcgtactttacatatatatttattagacaagaaaagcagattaaatagatatacattcgattaacgataagtaaaatgtaaaatcacaggattttcgtgtgtggtcttctacacagacaagatgaaacaattcggcattaatacctgagagcaggaagagcaagataaaaggtagtatttgttggcgatccccctagagtcttttacatcttcggaaaacaaaaactattttttctttaatttctttttttactttctatttttaatttatatatttatattaaaaaatttaaattataattatttttatagcacgtgatgaaaaggacccaggtggcacttttcggggaaatgtgcgcggaacccctatttgtttatttttctaaatacattcaaatatgtatccgctcatgagacaataaccctgataaatgcttcaataatattgaaaaaggaagagtatgagtattcaacatttccgtgtcgcccttattcccttttttgcggcattttgccttcctgtttttgctcacccagaaacgctggtgaaagtaaaagatgctgaagatcagttgggtgcacgagtgggttacatcgaactggatctcaacagcggtaagatccttgagagttttcgccccgaagaacgttttccaatgatgagcacttttaaagttctgctatgtggcgcggtattatcccgtattgacgccgggcaagagcaactcggtcgccgcatacactattctcagaatgacttggttgagtactcaccagtcacagaaaagcatcttacggatggcatgacagtaagagaattatgcagtgctgccataaccatgagtgataacactgcggccaacttacttctgacaacgatcggaggaccgaaggagctaaccgcttttttgcacaacatgggggatcatgtaactcgccttgatcgttgggaaccggagctgaatgaagccataccaaacgacgagcgtgacaccacgatgcctgtagcaatggcaacaacgttgcgcaaactattaactggcgaactacttactctagcttcccggcaacaattaatagactggatggaggcggataaagttgcaggaccacttctgcgctcggcccttccggctggctggtttattgctgataaatctggagccggtgagcgtgggtctcgcggtatcattgcagcactggggccagatggtaagccctcccgtatcgtagttatctacacgacggggagtcaggcaactatggatgaacgaaatagacagatcgctgagataggtgcctcactgattaagcattggtaactgtcagaccaagtttactcatatatactttagattgatttaaaacttcatttttaatttaaaaggatctaggtgaagatcctttttgataatctcatgaccaaaatcccttaacgtgagttttcgttccactgagcgtcagaccccgtagaaaagatcaaaggatcttcttgagatcctttttttctgcgcgtaatctgctgcttgcaaacaaaaaaaccaccgctaccagcggtggtttgtttgccggatcaagagctaccaactctttttccgaaggtaactggcttcagcagagcgcagataccaaatactgttcttctagtgtagccgtagttaggccaccacttcaagaactctgtagcaccgcctacatacctcgctctgctaatcctgttaccagtggctgctgccagtggcgataagtcgtgtcttaccgggttggactcaagacgatagttaccggataaggcgcagcggtcgggctgaacggggggttcgtgcacacagcccagcttggagcgaacgacctacaccgaactgagatacctacagcgtgagctatgagaaagcgccacgcttcccgaagggagaaaggcggacaggtatccggtaagcggcagggtcggaacaggagagcgcacgagggagcttccagggggaaacgcctggtatctttatagtcctgtcgggtttcgccacctctgacttgagcgtcgatttttgtgatgctcgtcaggggggcggagcctatggaaaaacgccagcaacgcggcctttttacggttcctggccttttgctggccttttgctcacatgttctttcctgcgttatcccctgattctgtggataaccgtattaccgcctttgagtgagctgataccgctcgccgcagccgaacgaccgagcgcagcgagtcagtgagcgaggaagcggaagagcgcccaatacgcaaaccgcctctccccgcgcgttggccgattcattaatgcagctggcacgacaggtttcccgactggaaagcgggcagtgagcgcaacgcaattaatgtgagttagctcactcattaggcaccccaggctttacactttatgcttccggctcgtatgttgtgtggaattgtgagcggataacaatttcacacaggaaacagctatgaccatgattacgccaagctcgaaattaaccctcactaaagggaacaaaagctggtaccaattccttgaattttcaaaaattcttactttttttttggatggacgcaaagaagtttaataatcatattacatggcattaccaccatatacatatccatatctaatcttacttatatgttgtggaaatgtaaagagccccattatcttagcctaaaaaaaccttctctttggaactttcagtaatacgcttaactgctcattgctatattgaagta

SEQ ID NO: 12 - DNA, 7547 bp, synthetic construct
  misc_feature 1..7547: note = Plasmid PW32; note (original language) = Plásmido PW32
  source 1..7547: mol_type = other DNA
cggattagaagccgccgagcgggtgacagccctccgaaggaagactctcctccgtgcgtcctcgtcttcaccggtcgcgttcctgaaacgcagatgtgcctcgcgccgcactgctccgaacaataaagattctacaatactagcttttatggttatgaagaggaaaaattggcagtaacctggccccacaaaccttcaaatgaacgaatcaaattaacaaccataggatgataatgcgattagttttttagccttatttctggggtaattaatcagcgaagcgatgatttttgatctattaacagatatataaatgcaaaaactgcataaccactttaactaatactttcaacattttcggtttgtattacttcttattcaaatgtaataaaagtatcaacaaaaaattgttaatatacctctatactttaacgtcaaggagaaaaaaccccggatcgaattccctacttcatacattttcaattaagatgcagttacttcgctgtttttcaatattttctgttattgcttcagttttagcacaggaactgacaactatatgcgagcaaatcccctcaccaactttagaatcgacgccgtactctttgtcaacgactactattttggccaacgggaaggcaatgcaaggagtttttgaatattacaaatcagtaacgtttgtcagtaattgcggttctcacccctcaacaactagcaaaggcagccccataaacacacagtatgtttttaaggacaatagctcgacgattgaaggtagatacccatacgacgttccagactacgctctgcaggctagtggtggaggaggctctggtggaggcggtagcggaggcggagggtcggctagctgcggtggcggcggtactagcaaaatttctcattttttgaaaatggaatctttgaattttattagagctcatactccatatattaatatttacaattgtgaaccagctaatccatctgaaaaaaattctccatctactcaatattgttattctattcaatcttcccaggtcgactgcgggggcggatccgaacaaaagcttatttctgaagaggacttgcaccaccaccaccaccactgactcgagatctgataacaacagtgtagatgtaacaaaatcgactttgttcccactgtacttttagctcgtacaaaatacaatatacttttcatttctccgtaaacaacatgttttcccatgtaatatccttttctatttttcgttccgttaccaactttacacatactttatatagctattcacttctatacactaaaaaactaagacaattttaattttgctgcctgccatatttcaatttgttataaattcctataatttatcctattagtagctaaaaaaagatgaatgtgaatcgaatcctaagagaattgagctccaattcgccctatagtgagtcgtattacaattcactggccgtcgttttacaacgtcgtgactgggaaaaccctggcgttacccaacttaatcgccttgcagcacatccccctttcgccagctggcgtaatagcgaagaggcccgcaccgatcgcctttcccaacagttgcgcagcctgaatggcgaatggacgcgccctgtagcggcgcattaagcgcggcgggtgtggtggttacgcgcagcgtgaccgctacacttgccagcgccctagcgcccgctcctttcgctttcttcccttcctttctcgccacgttcgccggctttccccgtcaagctctaaatcgggggctccctttagggttccgatttagtgctttacggcacctcgaccccaaaaaacttgattagggtgatggttcacgtagtgggccatcgccctgatagacggtttttcgccctttgacgttggagtccacgttctttaatagtggactcttgttccaaactggaacaacactcaaccctatctcggtctattcttttgatttataagggattttgccgatttcggcctattggttaaaaaatgagctgatttaacaaaaatttaacgcgaattttaacaaaatattaacgcttacaatttcctgatgcggtattttctccttacgcatctgtgcggtatttcacaccgcatatcgaccggtcgaggagaacttctagtatatctacatacctaatattattgccttattaaaaatggaatcccaacaattacatcaaaatccacattctcttcaaaatcaattgtcctgtacttccttgttcatgtgtgttcaaaaacgttatatttataggataattatactctatttctcaacaagtaattggttgtttggccgagcggtctaaggcgcctgattcaagaaatatcttgaccgcagttaactgtgggaatactcaggtatcgtaagatgcaagagttcgaatctcttagcaaccattatttttttcctcaacataacgagaacacacaggggcgctatcgcacagaatcaaattcgatgactggaaattttttgttaatttcagaggtcgcctgacgcatatacctttttcaactgaaaaattgggagaaaaaggaaaggtgagagcgccggaaccggcttttcatatagaatagagaagcgttcatgactaaatgcttgcatcacaatacttgaagttgacaatattatttaaggacctattgttttttccaataggtggttagcaatcgtcttactttctaacttttcttaccttttacatttcagcaatatatatatatatatttcaaggatataccattctaatgtctgcccctaagaagatcgtcgttttgccaggtgaccacgttggtcaagaaatcacagccgaagccattaaggttcttaaagctatttctgatgttcgttccaatgtcaagttcgatttcgaaaatcatttaattggtggtgctgctatcgatgctacaggtgttccacttccagatgaggcgctggaagcctccaagaaggctgatgccgttttgttaggtgctgtgggtggtcctaaatggggtaccggtagtgttagacctgaacaaggtttactaaaaatccgtaaagaacttcaattgtacgccaacttaagaccatgtaactttgcatccgactctcttttagacttatctccaatcaagccacaatttgctaaaggtactgacttcgttgttgtcagagaattagtgggaggtatttactttggtaagagaaaggaagacgatggtgatggtgtcgcttgggatagtgaacaatacaccgttccagaagtgcaaagaatcacaagaatggccgctttcatggccctacaacatgagccaccattgcctatttggtccttggataaagctaatgttttggcctcttcaagattatggagaaaaactgtggaggaaaccatcaagaacgaattccctacattgaaggttcaacatcaattgattgattctgccgccatgatcctagttaagaacccaacccacctaaatggtattataatcaccagcaacatgtttggtgatatcatctccgatgaagcctccgttatcccaggttccttgggtttgttgccatctgcgtccttggcctctttgccagacaagaacaccgcatttggtttgtacgaaccatgccacggttctgctccagatttgccaaagaataaggtcaaccctatcgccactatcttgtctgctgcaatgatgttgaaattgtcattgaacttgcctgaagaaggtaaggccattgaagatgcagttaaaaaggttttggatgcaggtatcagaactggtgatttaggtggttccaacagtaccaccgaagtcggtgatgctgtcgccgaagaagttaagaaaatccttgcttaaaaagattctctttttttatgatatttgtacataaactttataaatgaaattcataatagaaacgacacgaaattacaaaatggaatatgttcatagggtagacgaaactatatacgcaatctacatacatttatcaagaaggagaaaaaggaggatgtaaaggaatacaggtaagcaaattgatactaatggctcaacgtgataaggaaaaagaattgcactttaacattaatattgacaaggaggagggcaccacacaaaaagttaggtgtaacagaaaatcatgaaactatgattcctaatttatatattggaggattttctctaaaaaaaaaaaaatacaacaaataaaaaacactcaatgacctgaccatttgatggagtttaagtcaataccttcttgaaccatttcccataatggtgaaagttccctcaagaattttactctgtcagaaacggccttaacgacgtagtcgatatggtgcactctcagtacaatctgctctgatgccgcatagttaagccagccccgacacccgccaacacccgctgacgcgccctgacgggcttgtctgctcccggcatccgcttacagacaagctgtgaccgtctccgggagctgcatgtgtcagaggttttcaccgtcatcaccgaaacgcgcgagacgaaagggcctcgtgatacgcctatttttataggttaatgtcatgataataatggtttcttagacggatcgcttgcctgtaacttacacgcgcctcgtatcttttaatgatggaataatttgggaatttactctgtgtttatttatttttatgttttgtatttggattttagaaagtaaataaagaaggtagaagagttacggaatgaagaaaaaaaaataaacaaaggtttaaaaaatttcaacaaaaagcgtactttacatatatatttattagacaagaaaagcagattaaatagatatacattcgattaacgataagtaaaatgtaaaatcacaggattttcgtgtgtggtcttctacacagacaagatgaaacaattcggcattaatacctgagagcaggaagagcaagataaaaggtagtatttgttggcgatccccctagagtcttttacatcttcggaaaacaaaaactattttttctttaatttctttttttactttctatttttaatttatatatttatattaaaaaatttaaattataattatttttatagcacgtgatgaaaaggacccaggtggcacttttcggggaaatgtgcgcggaacccctatttgtttatttttctaaatacattcaaatatgtatccgctcatgagacaataaccctgataaatgcttcaataatattgaaaaaggaagagtatgagtattcaacatttccgtgtcgcccttattcccttttttgcggcattttgccttcctgtttttgctcacccagaaacgctggtgaaagtaaaagatgctgaagatcagttgggtgcacgagtgggttacatcgaactggatctcaacagcggtaagatccttgagagttttcgccccgaagaacgttttccaatgatgagcacttttaaagttctgctatgtggcgcggtattatcccgtattgacgccgggcaagagcaactcggtcgccgcatacactattctcagaatgacttggttgagtactcaccagtcacagaaaagcatcttacggatggcatgacagtaagagaattatgcagtgctgccataaccatgagtgataacactgcggccaacttacttctgacaacgatcggaggaccgaaggagctaaccgcttttttgcacaacatgggggatcatgtaactcgccttgatcgttgggaaccggagctgaatgaagccataccaaacgacgagcgtgacaccacgatgcctgtagcaatggcaacaacgttgcgcaaactattaactggcgaactacttactctagcttcccggcaacaattaatagactggatggaggcggataaagttgcaggaccacttctgcgctcggcccttccggctggctggtttattgctgataaatctggagccggtgagcgtgggtctcgcggtatcattgcagcactggggccagatggtaagccctcccgtatcgtagttatctacacgacggggagtcaggcaactatggatgaacgaaatagacagatcgctgagataggtgcctcactgattaagcattggtaactgtcagaccaagtttactcatatatactttagattgatttaaaacttcatttttaatttaaaaggatctaggtgaagatcctttttgataatctcatgaccaaaatcccttaacgtgagttttcgttccactgagcgtcagaccccgtagaaaagatcaaaggatcttcttgagatcctttttttctgcgcgtaatctgctgcttgcaaacaaaaaaaccaccgctaccagcggtggtttgtttgccggatcaagagctaccaactctttttccgaaggtaactggcttcagcagagcgcagataccaaatactgttcttctagtgtagccgtagttaggccaccacttcaagaactctgtagcaccgcctacatacctcgctctgctaatcctgttaccagtggctgctgccagtggcgataagtcgtgtcttaccgggttggactcaagacgatagttaccggataaggcgcagcggtcgggctgaacggggggttcgtgcacacagcccagcttggagcgaacgacctacaccgaactgagatacctacagcgtgagctatgagaaagcgccacgcttcccgaagggagaaaggcggacaggtatccggtaagcggcagggtcggaacaggagagcgcacgagggagcttccagggggaaacgcctggtatctttatagtcctgtcgggtttcgccacctctgacttgagcgtcgatttttgtgatgctcgtcaggggggcggagcctatggaaaaacgccagcaacgcggcctttttacggttcctggccttttgctggccttttgctcacatgttctttcctgcgttatcccctgattctgtggataaccgtattaccgcctttgagtgagctgataccgctcgccgcagccgaacgaccgagcgcagcgagtcagtgagcgaggaagcggaagagcgcccaatacgcaaaccgcctctccccgcgcgttggccgattcattaatgcagctggcacgacaggtttcccgactggaaagcgggcagtgagcgcaacgcaattaatgtgagttagctcactcattaggcaccccaggctttacactttatgcttccggctcgtatgttgtgtggaattgtgagcggataacaatttcacacaggaaacagctatgaccatgattacgccaagctcgaaattaaccctcactaaagggaacaaaagctggtaccaattccttgaattttcaaaaattcttactttttttttggatggacgcaaagaagtttaataatcatattacatggcattaccaccatatacatatccatatctaatcttacttatatgttgtggaaatgtaaagagccccattatcttagcctaaaaaaaccttctctttggaactttcagtaatacgcttaactgctcattgctatattgaagta

SEQ ID NO: 13 - DNA, 6356 bp, synthetic construct
  misc_feature 1..6356: note = Plasmid PW33; note (original language) = Plásmido PW33
  source 1..6356: mol_type = other DNA
cggattagaagccgccgagcgggtgacagccctccgaaggaagactctcctccgtgcgtcctcgtcttcaccggtcgcgttcctgaaacgcagatgtgcctcgcgccgcactgctccgaacaataaagattctacaatactagcttttatggttatgaagaggaaaaattggcagtaacctggccccacaaaccttcaaatgaacgaatcaaattaacaaccataggatgataatgcgattagttttttagccttatttctggggtaattaatcagcgaagcgatgatttttgatctattaacagatatataaatgcaaaaactgcataaccactttaactaatactttcaacattttcggtttgtattacttcttattcaaatgtaataaaagtatcaacaaaaaattgttaatatacctctatactttaacgtcaaggagaaaaaaccccggatcgaattccctacttcatacattttcaattaagatgcagttacttcgctgtttttcaatattttctgttattgcttcagttttagcacaggaactgacaactatatgcgagcaaatcccctcaccaactttagaatcgacgccgtactctttgtcaacgactactattttggccaacgggaaggcaatgcaaggagtttttgaatattacaaatcagtaacgtttgtcagtaattgcggttctcacccctcaacaactagcaaaggcagccccataaacacacagtatgtttttaaggacaatagctcgacgattgaaggtagatacccatacgacgttccagactacgctctgcaggaaaatttgtattttcaatctctgcaggctagtggtggaggaggctctggtggaggcggtagcggaggcggagggtcggctagctgcggtggcggcggtactagcaaaatttctcattttttgaaaatggaatctttgaattttattagagctcatactccatatattaatatttacaattgtgaaccagctaatccatctgaaaaaaattctccatctactcaatattgttattctattcaatcttcccaggtcgactgcgggggcggatccgaacaaaagcttatttctgaagaggacttgcaccaccaccaccaccactgactcgagatctgataacaacagtgtagatgtaacaaaatcgactttgttcccactgtacttttagctcgtacaaaatacaatatacttttcatttctccgtaaacaacatgttttcccatgtaatatccttttctatttttcgttccgttaccaactttacacatactttatatagctattcacttctatacactaaaaaactaagacaattttaattttgctgcctgccatatttcaatttgttataaattcctataatttatcctattagtagctaaaaaaagatgaatgtgaatcgaatcctaagagaattgagctccaattcgccctatagtgagtcgtattacaattcactggccgtcgttttacaacgtcgtgactgggaaaaccctggcgttacccaacttaatcgccttgcagcacatccccctttcgccagctggcgtaatagcgaagaggcccgcaccgatcgcctttcccaacagttgcgcagcctgaatggcgaatggacgcgccctgtagcggcgcattaagcgcggcgggtgtggtggttacgcgcagcgtgaccgctacacttgccagcgccctagcgcccgctcctttcgctttcttcccttcctttctcgccacgttcgccggctttccccgtcaagctctaaatcgggggctccctttagggttccgatttagtgctttacggcacctcgaccccaaaaaacttgattagggtgatggttcacgtagtgggccatcgccctgatagacggtttttcgccctttgacgttggagtccacgttctttaatagtggactcttgttccaaactggaacaacactcaaccctatctcggtctattcttttgatttataagggattttgccgatttcggcctattggttaaaaaatgagctgatttaacaaaaatttaacgcgaattttaacaaaatattaacgcttacaatttcctgatgcggtattttctccttacgcatctgtgcggtatttcacaccgcatagatcggcaagtgcacaaacaatacttaaataaatactactcagtaataacctatttcttagcatttttgacgaaatttgctattttgttagagtcttttacaccatttgtctccacacctccgcttacatcaacaccaataacgccatttaatctaagcgcatcaccaacattttctggcgtcagtccaccagctaacataaaatgtaagctttcggggctctcttgccttccaacccagtcagaaatcgagttccaatccaaaagttcacctgtcccacctgcttctgaatcaaacaagggaataaacgaatgaggtttctgtgaagctgcactgagtagtatgttgcagtcttttggaaatacgagtcttttaataactggcaaaccgaggaactcttggtattcttgccacgactcatctccatgcagttggacgatatcaatgccgtaatcattgaccagagccaaaacatcctccttaggttgattacgaaacacgccaaccaagtatttcggagtgcctgaactatttttatatgcttttacaagacttgaaattttccttgcaataaccgggtcaattgttctctttctattgggcacacatataatacccagcaagtcagcatcggaatctagagcacattctgcggcctctgtgctctgcaagccgcaaactttcaccaatggaccagaactacctgtgaaattaataacagacatactccaagctgcctttgtgtgcttaatcacgtatactcacgtgctcaatagtcaccaatgccctccctcttggccctctccttttcttttttcgaccgaattaattcttaatcggcaaaaaaagaaaagctccggatcaagattgtacgtaaggtgacaagctatttttcaataaagaatatcttccactactgccatctggcgtcataactgcaaagtacacatatattacgatgctgttctattaaatgcttcctatattatatatatagtaatgtcgtgatctatggtgcactctcagtacaatctgctctgatgccgcatagttaagccagccccgacacccgccaacacccgctgacgcgccctgacgggcttgtctgctcccggcatccgcttacagacaagctgtgaccgtctccgggagctgcatgtgtcagaggttttcaccgtcatcaccgaaacgcgcgagacgaaagggcctcgtgatacgcctatttttataggttaatgtcatgataataatggtttcttagacggatcgcttgcctgtaacttacacgcgcctcgtatcttttaatgatggaataatttgggaatttactctgtgtttatttatttttatgttttgtatttggattttagaaagtaaataaagaaggtagaagagttacggaatgaagaaaaaaaaataaacaaaggtttaaaaaatttcaacaaaaagcgtactttacatatatatttattagacaagaaaagcagattaaatagatatacattcgattaacgataagtaaaatgtaaaatcacaggattttcgtgtgtggtcttctacacagacaagatgaaacaattcggcattaatacctgagagcaggaagagcaagataaaaggtagtatttgttggcgatccccctagagtcttttacatcttcggaaaacaaaaactattttttctttaatttctttttttactttctatttttaatttatatatttatattaaaaaatttaaattataattatttttatagcacgtgatgaaaaggacccaggtggcacttttcggggaaatgtgcgcggaacccctatttgtttatttttctaaatacattcaaatatgtatccgctcatgagacaataaccctgataaatgcttcaataatattgaaaaaggaagagtatgagtattcaacatttccgtgtcgcccttattcccttttttgcggcattttgccttcctgtttttgctcacccagaaacgctggtgaaagtaaaagatgctgaagatcagttgggtgcacgagtgggttacatcgaactggatctcaacagcggtaagatccttgagagttttcgccccgaagaacgttttccaatgatgagcacttttaaagttctgctatgtggcgcggtattatcccgtattgacgccgggcaagagcaactcggtcgccgcatacactattctcagaatgacttggttgagtactcaccagtcacagaaaagcatcttacggatggcatgacagtaagagaattatgcagtgctgccataaccatgagtgataacactgcggccaacttacttctgacaacgatcggaggaccgaaggagctaaccgcttttttgcacaacatgggggatcatgtaactcgccttgatcgttgggaaccggagctgaatgaagccataccaaacgacgagcgtgacaccacgatgcctgtagcaatggcaacaacgttgcgcaaactattaactggcgaactacttactctagcttcccggcaacaattaatagactggatggaggcggataaagttgcaggaccacttctgcgctcggcccttccggctggctggtttattgctgataaatctggagccggtgagcgtgggtctcgcggtatcattgcagcactggggccagatggtaagccctcccgtatcgtagttatctacacgacggggagtcaggcaactatggatgaacgaaatagacagatcgctgagataggtgcctcactgattaagcattggtaactgtcagaccaagtttactcatatatactttagattgatttaaaacttcatttttaatttaaaaggatctaggtgaagatcctttttgataatctcatgaccaaaatcccttaacgtgagttttcgttccactgagcgtcagaccccgtagaaaagatcaaaggatcttcttgagatcctttttttctgcgcgtaatctgctgcttgcaaacaaaaaaaccaccgctaccagcggtggtttgtttgccggatcaagagctaccaactctttttccgaaggtaactggcttcagcagagcgcagataccaaatactgttcttctagtgtagccgtagttaggccaccacttcaagaactctgtagcaccgcctacatacctcgctctgctaatcctgttaccagtggctgctgccagtggcgataagtcgtgtcttaccgggttggactcaagacgatagttaccggataaggcgcagcggtcgggctgaacggggggttcgtgcacacagcccagcttggagcgaacgacctacaccgaactgagatacctacagcgtgagctatgagaaagcgccacgcttcccgaagggagaaaggcggacaggtatccggtaagcggcagggtcggaacaggagagcgcacgagggagcttccagggggaaacgcctggtatctttatagtcctgtcgggtttcgccacctctgacttgagcgtcgatttttgtgatgctcgtcaggggggcggagcctatggaaaaacgccagcaacgcggcctttttacggttcctggccttttgctggccttttgctcacatgttctttcctgcgttatcccctgattctgtggataaccgtattaccgcctttgagtgagctgataccgctcgccgcagccgaacgaccgagcgcagcgagtcagtgagcgaggaagcggaagagcgcccaatacgcaaaccgcctctccccgcgcgttggccgattcattaatgcagctggcacgacaggtttcccgactggaaagcgggcagtgagcgcaacgcaattaatgtgagttagctcactcattaggcaccccaggctttacactttatgcttccggctcgtatgttgtgtggaattgtgagcggataacaatttcacacaggaaacagctatgaccatgattacgccaagctcgaaattaaccctcactaaagggaacaaaagctggtaccaattccttgaattttcaaaaattcttactttttttttggatggacgcaaagaagtttaataatcatattacatggcattaccaccatatacatatccatatctaatcttacttatatgttgtggaaatgtaaagagccccattatcttagcctaaaaaaaccttctctttggaactttcagtaatacgcttaactgctcattgctatattgaagta

SEQ ID NO: 14 - DNA, 6530 bp, synthetic construct
  misc_feature 1..6530: note = Plasmid PW34; note (original language) = Plásmido PW34
  source 1..6530: mol_type = other DNA
cggattagaagccgccgagcgggtgacagccctccgaaggaagactctcctccgtgcgtcctcgtcttcaccggtcgcgttcctgaaacgcagatgtgcctcgcgccgcactgctccgaacaataaagattctacaatactagcttttatggttatgaagaggaaaaattggcagtaacctggccccacaaaccttcaaatgaacgaatcaaattaacaaccataggatgataatgcgattagttttttagccttatttctggggtaattaatcagcgaagcgatgatttttgatctattaacagatatataaatgcaaaaactgcataaccactttaactaatactttcaacattttcggtttgtattacttcttattcaaatgtaataaaagtatcaacaaaaaattgttaatatacctctatactttaacgtcaaggagaaaaaaccccggatcgaattccctacttcatacattttcaattaagatgcagttacttcgctgtttttcaatattttctgttattgcttcagttttagcacaggaactgacaactatatgcgagcaaatcccctcaccaactttagaatcgacgccgtactctttgtcaacgactactattttggccaacgggaaggcaatgcaaggagtttttgaatattacaaatcagtaacgtttgtcagtaattgcggttctcacccctcaacaactagcaaaggcagccccataaacacacagtatgtttttaaggacaatagctcgacgattgaaggtagatacccatacgacgttccagactacgctctgcaggaaaatttgtattttcaatctctgcaggctagtggtggaggaggctctggtggaggcggtagcggaggcggagggtcggctagctgcggtggcggcggtactagcaaaatttctcattttttgaaaatggaatctttgaattttattagagctcatactccatatattaatatttacaattgtgaaccagctaatccatctgaaaaaaattctccatctactcaatattgttattctattcaatcttcccaggtcgactgcgggggcggatccgaacaaaagcttatttctgaagaggacttgcaccaccaccaccaccactgactcgagatctgataacaacagtgtagatgtaacaaaatcgactttgttcccactgtacttttagctcgtacaaaatacaatatacttttcatttctccgtaaacaacatgttttcccatgtaatatccttttctatttttcgttccgttaccaactttacacatactttatatagctattcacttctatacactaaaaaactaagacaattttaattttgctgcctgccatatttcaatttgttataaattcctataatttatcctattagtagctaaaaaaagatgaatgtgaatcgaatcctaagagaattgagctccaattcgccctatagtgagtcgtattacaattcactggccgtcgttttacaacgtcgtgactgggaaaaccctggcgttacccaacttaatcgccttgcagcacatccccctttcgccagctggcgtaatagcgaagaggcccgcaccgatcgcctttcccaacagttgcgcagcctgaatggcgaatggacgcgccctgtagcggcgcattaagcgcggcgggtgtggtggttacgcgcagcgtgaccgctacacttgccagcgccctagcgcccgctcctttcgctttcttcccttcctttctcgccacgttcgccggctttccccgtcaagctctaaatcgggggctccctttagggttccgatttagtgctttacggcacctcgaccccaaaaaacttgattagggtgatggttcacgtagtgggccatcgccctgatagacggtttttcgccctttgacgttggagtccacgttctttaatagtggactcttgttccaaactggaacaacactcaaccctatctcggtctattcttttgatttataagggattttgccgatttcggcctattggttaaaaaatgagctgatttaacaaaaatttaacgcgaattttaacaaaatattaacgtttacaatttcctgatgcggtattttctccttacgcatctgtgcggtatttcacaccgcatagatccgtcgagttcaagagaaaaaaaaagaaaaagcaaaaagaaaaaaggaaagcgcgcctcgttcagaatgacacgtatagaatgatgcattaccttgtcatcttcagtatcatactgttcgtatacatacttactgacattcataggtatacatatatacacatgtatatatatcgtatgctgcagctttaaataatcggtgtcactacataagaacacctttggtggagggaacatcgttggtaccattgggcgaggtggcttctcttatggcaaccgcaagagccttgaacgcactctcactacggtgatgatcattcttgcctcgcagacaatcaacgtggagggtaattctgctagcctctgcaaagctttcaagaaaatgcgggatcatctcgcaagagagatctcctactttctccctttgcaaaccaagttcgacaactgcgtacggcctgttcgaaagatctaccaccgctctggaaagtgcctcatccaaaggcgcaaatcctgatccaaacctttttactccacgcgccagtagggcctctttaaaagcttgaccgagagcaatcccgcagtcttcagtggtgtgatggtcgtctatgtgtaagtcaccaatgcactcaacgattagcgaccagccggaatgcttggccagagcatgtatcatatggtccagaaaccctatacctgtgtggacgttaatcacttgcgattgtgtggcctgttctgctactgcttctgcctctttttctgggaagatcgagtgctctatcgctaggggaccaccctttaaagagatcgcaatctgaatcttggtttcatttgtaatacgctttactagggctttctgctctgtcatctttgccttcgtttatcttgcctgctcattttttagtatattcttcgaagaaatcacattactttatataatgtataattcattatgtgataatgccaatcgctaagaaaaaaaaagagtcatccgctaggggaaaaaaaaaaatgaaaatcattaccgaggcataaaaaaatatagagtgtactagaggaggccaagagtaatagaaaaagaaaattgcgggaaaggactgtgttatgacttccctgactaatgccgtgttcaaacgatacctggcagtgactcctagcgctcaccaagctcttaaaacgggaatttatggtgcactctcagtacaatctgctctgatgccgcatagttaagccagccccgacacccgccaacacccgctgacgcgccctgacgggcttgtctgctcccggcatccgcttacagacaagctgtgaccgtctccgggagctgcatgtgtcagaggttttcaccgtcatcaccgaaacgcgcgagacgaaagggcctcgtgatacgcctatttttataggttaatgtcatgataataatggtttcttagacggatcgcttgcctgtaacttacacgcgcctcgtatcttttaatgatggaataatttgggaatttactctgtgtttatttatttttatgttttgtatttggattttagaaagtaaataaagaaggtagaagagttacggaatgaagaaaaaaaaataaacaaaggtttaaaaaatttcaacaaaaagcgtactttacatatatatttattagacaagaaaagcagattaaatagatatacattcgattaacgataagtaaaatgtaaaatcacaggattttcgtgtgtggtcttctacacagacaagatgaaacaattcggcattaatacctgagagcaggaagagcaagataaaaggtagtatttgttggcgatccccctagagtcttttacatcttcggaaaacaaaaactattttttctttaatttctttttttactttctatttttaatttatatatttatattaaaaaatttaaattataattatttttatagcacgtgatgaaaaggacccaggtggcacttttcggggaaatgtgcgcggaacccctatttgtttatttttctaaatacattcaaatatgtatccgctcatgagacaataaccctgataaatgcttcaataatattgaaaaaggaagagtatgagtattcaacatttccgtgtcgcccttattcccttttttgcggcattttgccttcctgtttttgctcacccagaaacgctggtgaaagtaaaagatgctgaagatcagttgggtgcacgagtgggttacatcgaactggatctcaacagcggtaagatccttgagagttttcgccccgaagaacgttttccaatgatgagcacttttaaagttctgctatgtggcgcggtattatcccgtattgacgccgggcaagagcaactcggtcgccgcatacactattctcagaatgacttggttgagtactcaccagtcacagaaaagcatcttacggatggcatgacagtaagagaattatgcagtgctgccataaccatgagtgataacactgcggccaacttacttctgacaacgatcggaggaccgaaggagctaaccgcttttttgcacaacatgggggatcatgtaactcgccttgatcgttgggaaccggagctgaatgaagccataccaaacgacgagcgtgacaccacgatgcctgtagcaatggcaacaacgttgcgcaaactattaactggcgaactacttactctagcttcccggcaacaattaatagactggatggaggcggataaagttgcaggaccacttctgcgctcggcccttccggctggctggtttattgctgataaatctggagccggtgagcgtgggtctcgcggtatcattgcagcactggggccagatggtaagccctcccgtatcgtagttatctacacgacggggagtcaggcaactatggatgaacgaaatagacagatcgctgagataggtgcctcactgattaagcattggtaactgtcagaccaagtttactcatatatactttagattgatttaaaacttcatttttaatttaaaaggatctaggtgaagatcctttttgataatctcatgaccaaaatcccttaacgtgagttttcgttccactgagcgtcagaccccgtagaaaagatcaaaggatcttcttgagatcctttttttctgcgcgtaatctgctgcttgcaaacaaaaaaaccaccgctaccagcggtggtttgtttgccggatcaagagctaccaactctttttccgaaggtaactggcttcagcagagcgcagataccaaatactgttcttctagtgtagccgtagttaggccaccacttcaagaactctgtagcaccgcctacatacctcgctctgctaatcctgttaccagtggctgctgccagtggcgataagtcgtgtcttaccgggttggactcaagacgatagttaccggataaggcgcagcggtcgggctgaacggggggttcgtgcacacagcccagcttggagcgaacgacctacaccgaactgagatacctacagcgtgagctatgagaaagcgccacgcttcccgaagggagaaaggcggacaggtatccggtaagcggcagggtcggaacaggagagcgcacgagggagcttccagggggaaacgcctggtatctttatagtcctgtcgggtttcgccacctctgacttgagcgtcgatttttgtgatgctcgtcaggggggcggagcctatggaaaaacgccagcaacgcggcctttttacggttcctggccttttgctggccttttgctcacatgttctttcctgcgttatcccctgattctgtggataaccgtattaccgcctttgagtgagctgataccgctcgccgcagccgaacgaccgagcgcagcgagtcagtgagcgaggaagcggaagagcgcccaatacgcaaaccgcctctccccgcgcgttggccgattcattaatgcagctggcacgacaggtttcccgactggaaagcgggcagtgagcgcaacgcaattaatgtgagttagctcactcattaggcaccccaggctttacactttatgcttccggctcgtatgttgtgtggaattgtgagcggataacaatttcacacaggaaacagctatgaccatgattacgccaagctcgaaattaaccctcactaaagggaacaaaagctggtaccaattccttgaattttcaaaaattcttactttttttttggatggacgcaaagaagtttaataatcatattacatggcattaccaccatatacatatccatatctaatcttacttatatgttgtggaaatgtaaagagccccattatcttagcctaaaaaaaccttctctttggaactttcagtaatacgcttaactgctcattgctatattgaagta

SEQ ID NO: 15 - DNA, 7574 bp, synthetic construct
  misc_feature 1..7574: note = Plasmid PW35; note (original language) = Plásmido PW35
  source 1..7574: mol_type = other DNA
cggattagaagccgccgagcgggtgacagccctccgaaggaagactctcctccgtgcgtcctcgtcttcaccggtcgcgttcctgaaacgcagatgtgcctcgcgccgcactgctccgaacaataaagattctacaatactagcttttatggttatgaagaggaaaaattggcagtaacctggccccacaaaccttcaaatgaacgaatcaaattaacaaccataggatgataatgcgattagttttttagccttatttctggggtaattaatcagcgaagcgatgatttttgatctattaacagatatataaatgcaaaaactgcataaccactttaactaatactttcaacattttcggtttgtattacttcttattcaaatgtaataaaagtatcaacaaaaaattgttaatatacctctatactttaacgtcaaggagaaaaaaccccggatcgaattccctacttcatacattttcaattaagatgcagttacttcgctgtttttcaatattttctgttattgcttcagttttagcacaggaactgacaactatatgcgagcaaatcccctcaccaactttagaatcgacgccgtactctttgtcaacgactactattttggccaacgggaaggcaatgcaaggagtttttgaatattacaaatcagtaacgtttgtcagtaattgcggttctcacccctcaacaactagcaaaggcagccccataaacacacagtatgtttttaaggacaatagctcgacgattgaaggtagatacccatacgacgttccagactacgctctgcaggaaaatttgtattttcaatctctgcaggctagtggtggaggaggctctggtggaggcggtagcggaggcggagggtcggctagctgcggtggcggcggtactagcaaaatttctcattttttgaaaatggaatctttgaattttattagagctcatactccatatattaatatttacaattgtgaaccagctaatccatctgaaaaaaattctccatctactcaatattgttattctattcaatcttcccaggtcgactgcgggggcggatccgaacaaaagcttatttctgaagaggacttgcaccaccaccaccaccactgactcgagatctgataacaacagtgtagatgtaacaaaatcgactttgttcccactgtacttttagctcgtacaaaatacaatatacttttcatttctccgtaaacaacatgttttcccatgtaatatccttttctatttttcgttccgttaccaactttacacatactttatatagctattcacttctatacactaaaaaactaagacaattttaattttgctgcctgccatatttcaatttgttataaattcctataatttatcctattagtagctaaaaaaagatgaatgtgaatcgaatcctaagagaattgagctccaattcgccctatagtgagtcgtattacaattcactggccgtcgttttacaacgtcgtgactgggaaaaccctggcgttacccaacttaatcgccttgcagcacatccccctttcgccagctggcgtaatagcgaagaggcccgcaccgatcgcctttcccaacagttgcgcagcctgaatggcgaatggacgcgccctgtagcggcgcattaagcgcggcgggtgtggtggttacgcgcagcgtgaccgctacacttgccagcgccctagcgcccgctcctttcgctttcttcccttcctttctcgccacgttcgccggctttccccgtcaagctctaaatcgggggctccctttagggttccgatttagtgctttacggcacctcgaccccaaaaaacttgattagggtgatggttcacgtagtgggccatcgccctgatagacggtttttcgccctttgacgttggagtccacgttctttaatagtggactcttgttccaaactggaacaacactcaaccctatctcggtctattcttttgatttataagggattttgccgatttcggcctattggttaaaaaatgagctgatttaacaaaaatttaacgcgaattttaacaaaatattaacgcttacaatttcctgatgcggtattttctccttacgcatctgtgcggtatttcacaccgcatatcgaccggtcgaggagaacttctagtatatctacatacctaatattattgccttattaaaaatggaatcccaacaattacatcaaaatccacattctcttcaaaatcaattgtcctgtacttccttgttcatgtgtgttcaaaaacgttatatttataggataattatactctatttctcaacaagtaattggttgtttggccgagcggtctaaggcgcctgattcaagaaatatcttgaccgcagttaactgtgggaatactcaggtatcgtaagatgcaagagttcgaatctcttagcaaccattatttttttcctcaacataacgagaacacacaggggcgctatcgcacagaatcaaattcgatgactggaaattttttgttaatttcagaggtcgcctgacgcatatacctttttcaactgaaaaattgggagaaaaaggaaaggtgagagcgccggaaccggcttttcatatagaatagagaagcgttcatgactaaatgcttgcatcacaatacttgaagttgacaatattatttaaggacctattgttttttccaataggtggttagcaatcgtcttactttctaacttttcttaccttttacatttcagcaatatatatatatatatttcaaggatataccattctaatgtctgcccctaagaagatcgtcgttttgccaggtgaccacgttggtcaagaaatcacagccgaagccattaaggttcttaaagctatttctgatgttcgttccaatgtcaagttcgatttcgaaaatcatttaattggtggtgctgctatcgatgctacaggtgttccacttccagatgaggcgctggaagcctccaagaaggctgatgccgttttgttaggtgctgtgggtggtcctaaatggggtaccggtagtgttagacctgaacaaggtttactaaaaatccgtaaagaacttcaattgtacgccaacttaagaccatgtaactttgcatccgactctcttttagacttatctccaatcaagccacaatttgctaaaggtactgacttcgttgttgtcagagaattagtgggaggtatttactttggtaagagaaaggaagacgatggtgatggtgtcgcttgggatagtgaacaatacaccgttccagaagtgcaaagaatcacaagaatggccgctttcatggccctacaacatgagccaccattgcctatttggtccttggataaagctaatgttttggcctcttcaagattatggagaaaaactgtggaggaaaccatcaagaacgaattccctacattgaaggttcaacatcaattgattgattctgccgccatgatcctagttaagaacccaacccacctaaatggtattataatcaccagcaacatgtttggtgatatcatctccgatgaagcctccgttatcccaggttccttgggtttgttgccatctgcgtccttggcctctttgccagacaagaacaccgcatttggtttgtacgaaccatgccacggttctgctccagatttgccaaagaataaggtcaaccctatcgccactatcttgtctgctgcaatgatgttgaaattgtcattgaacttgcctgaagaaggtaaggccattgaagatgcagttaaaaaggttttggatgcaggtatcagaactggtgatttaggtggttccaacagtaccaccgaagtcggtgatgctgtcgccgaagaagttaagaaaatccttgcttaaaaagattctctttttttatgatatttgtacataaactttataaatgaaattcataatagaaacgacacgaaattacaaaatggaatatgttcatagggtagacgaaactatatacgcaatctacatacatttatcaagaaggagaaaaaggaggatgtaaaggaatacaggtaagcaaattgatactaatggctcaacgtgataaggaaaaagaattgcactttaacattaatattgacaaggaggagggcaccacacaaaaagttaggtgtaacagaaaatcatgaaactatgattcctaatttatatattggaggattttctctaaaaaaaaaaaaatacaacaaataaaaaacactcaatgacctgaccatttgatggagtttaagtcaataccttcttgaaccatttcccataatggtgaaagttccctcaagaattttactctgtcagaaacggccttaacgacgtagtcgatatggtgcactctcagtacaatctgctctgatgccgcatagttaagccagccccgacacccgccaacacccgctgacgcgccctgacgggcttgtctgctcccggcatccgcttacagacaagctgtgaccgtctccgggagctgcatgtgtcagaggttttcaccgtcatcaccgaaacgcgcgagacgaaagggcctcgtgatacgcctatttttataggttaatgtcatgataataatggtttcttagacggatcgcttgcctgtaacttacacgcgcctcgtatcttttaatgatggaataatttgggaatttactctgtgtttatttatttttatgttttgtatttggattttagaaagtaaataaagaaggtagaagagttacggaatgaagaaaaaaaaataaacaaaggtttaaaaaatttcaacaaaaagcgtactttacatatatatttattagacaagaaaagcagattaaatagatatacattcgattaacgataagtaaaatgtaaaatcacaggattttcgtgtgtggtcttctacacagacaagatgaaacaattcggcattaatacctgagagcaggaagagcaagataaaaggtagtatttgttggcgatccccctagagtcttttacatcttcggaaaacaaaaactattttttctttaatttctttttttactttctatttttaatttatatatttatattaaaaaatttaaattataattatttttatagcacgtgatgaaaaggacccaggtggcacttttcggggaaatgtgcgcggaacccctatttgtttatttttctaaatacattcaaatatgtatccgctcatgagacaataaccctgataaatgcttcaataatattgaaaaaggaagagtatgagtattcaacatttccgtgtcgcccttattcccttttttgcggcattttgccttcctgtttttgctcacccagaaacgctggtgaaagtaaaagatgctgaagatcagttgggtgcacgagtgggttacatcgaactggatctcaacagcggtaagatccttgagagttttcgccccgaagaacgttttccaatgatgagcacttttaaagttctgctatgtggcgcggtattatcccgtattgacgccgggcaagagcaactcggtcgccgcatacactattctcagaatgacttggttgagtactcaccagtcacagaaaagcatcttacggatggcatgacagtaagagaattatgcagtgctgccataaccatgagtgataacactgcggccaacttacttctgacaacgatcggaggaccgaaggagctaaccgcttttttgcacaacatgggggatcatgtaactcgccttgatcgttgggaaccggagctgaatgaagccataccaaacgacgagcgtgacaccacgatgcctgtagcaatggcaacaacgttgcgcaaactattaactggcgaactacttactctagcttcccggcaacaattaatagactggatggaggcggataaagttgcaggaccacttctgcgctcggcccttccggctggctggtttattgctgataaatctggagccggtgagcgtgggtctcgcggtatcattgcagcactggggccagatggtaagccctcccgtatcgtagttatctacacgacggggagtcaggcaactatggatgaacgaaatagacagatcgctgagataggtgcctcactgattaagcattggtaactgtcagaccaagtttactcatatatactttagattgatttaaaacttcatttttaatttaaaaggatctaggtgaagatcctttttgataatctcatgaccaaaatcccttaacgtgagttttcgttccactgagcgtcagaccccgtagaaaagatcaaaggatcttcttgagatcctttttttctgcgcgtaatctgctgcttgcaaacaaaaaaaccaccgctaccagcggtggtttgtttgccggatcaagagctaccaactctttttccgaaggtaactggcttcagcagagcgcagataccaaatactgttcttctagtgtagccgtagttaggccaccacttcaagaactctgtagcaccgcctacatacctcgctctgctaatcctgttaccagtggctgctgccagtggcgataagtcgtgtcttaccgggttggactcaagacgatagttaccggataaggcgcagcggtcgggctgaacggggggttcgtgcacacagcccagcttggagcgaacgacctacaccgaactgagatacctacagcgtgagctatgagaaagcgccacgcttcccgaagggagaaaggcggacaggtatccggtaagcggcagggtcggaacaggagagcgcacgagggagcttccagggggaaacgcctggtatctttatagtcctgtcgggtttcgccacctctgacttgagcgtcgatttttgtgatgctcgtcaggggggcggagcctatggaaaaacgccagcaacgcggcctttttacggttcctggccttttgctggccttttgctcacatgttctttcctgcgttatcccctgattctgtggataaccgtattaccgcctttgagtgagctgataccgctcgccgcagccgaacgaccgagcgcagcgagtcagtgagcgaggaagcggaagagcgcccaatacgcaaaccgcctctccccgcgcgttggccgattcattaatgcagctggcacgacaggtttcccgactggaaagcgggcagtgagcgcaacgcaattaatgtgagttagctcactcattaggcaccccaggctttacactttatgcttccggctcgtatgttgtgtggaattgtgagcggataacaatttcacacaggaaacagctatgaccatgattacgccaagctcgaaattaaccctcactaaagggaacaaaagctggtaccaattccttgaattttcaaaaattcttactttttttttggatggacgcaaagaagtttaataatcatattacatggcattaccaccatatacatatccatatctaatcttacttatatgttgtggaaatgtaaagagccccattatcttagcctaaaaaaaccttctctttggaactttcagtaatacgcttaactgctcattgctatattgaagta

SEQ ID NO: 16 - DNA, 6353 bp, synthetic construct
  misc_feature 1..6353: note = Plasmid PW36; note (original language) = Plásmido PW36
  source 1..6353: mol_type = other DNA
cggattagaagccgccgagcgggtgacagccctccgaaggaagactctcctccgtgcgtcctcgtcttcaccggtcgcgttcctgaaacgcagatgtgcctcgcgccgcactgctccgaacaataaagattctacaatactagcttttatggttatgaagaggaaaaattggcagtaacctggccccacaaaccttcaaatgaacgaatcaaattaacaaccataggatgataatgcgattagttttttagccttatttctggggtaattaatcagcgaagcgatgatttttgatctattaacagatatataaatgcaaaaactgcataaccactttaactaatactttcaacattttcggtttgtattacttcttattcaaatgtaataaaagtatcaacaaaaaattgttaatatacctctatactttaacgtcaaggagaaaaaaccccggatcgaattccctacttcatacattttcaattaagatgcagttacttcgctgtttttcaatattttctgttattgcttcagttttagcacaggaactgacaactatatgcgagcaaatcccctcaccaactttagaatcgacgccgtactctttgtcaacgactactattttggccaacgggaaggcaatgcaaggagtttttgaatattacaaatcagtaacgtttgtcagtaattgcggttctcacccctcaacaactagcaaaggcagccccataaacacacagtatgtttttaaggacaatagctcgacgattgaaggtagatacccatacgacgttccagactacgctctgcagttggttccaagaggttctctgcaggctagtggtggaggaggctctggtggaggcggtagcggaggcggagggtcggctagctgcggtggcggcggtactagcaaaatttctcattttttgaaaatggaatctttgaattttattagagctcatactccatatattaatatttacaattgtgaaccagctaatccatctgaaaaaaattctccatctactcaatattgttattctattcaatcttcccaggtcgactgcgggggcggatccgaacaaaagcttatttctgaagaggacttgcaccaccaccaccaccactgactcgagatctgataacaacagtgtagatgtaacaaaatcgactttgttcccactgtacttttagctcgtacaaaatacaatatacttttcatttctccgtaaacaacatgttttcccatgtaatatccttttctatttttcgttccgttaccaactttacacatactttatatagctattcacttctatacactaaaaaactaagacaattttaattttgctgcctgccatatttcaatttgttataaattcctataatttatcctattagtagctaaaaaaagatgaatgtgaatcgaatcctaagagaattgagctccaattcgccctatagtgagtcgtattacaattcactggccgtcgttttacaacgtcgtgactgggaaaaccctggcgttacccaacttaatcgccttgcagcacatccccctttcgccagctggcgtaatagcgaagaggcccgcaccgatcgcctttcccaacagttgcgcagcctgaatggcgaatggacgcgccctgtagcggcgcattaagcgcggcgggtgtggtggttacgcgcagcgtgaccgctacacttgccagcgccctagcgcccgctcctttcgctttcttcccttcctttctcgccacgttcgccggctttccccgtcaagctctaaatcgggggctccctttagggttccgatttagtgctttacggcacctcgaccccaaaaaacttgattagggtgatggttcacgtagtgggccatcgccctgatagacggtttttcgccctttgacgttggagtccacgttctttaatagtggactcttgttccaaactggaacaacactcaaccctatctcggtctattcttttgatttataagggattttgccgatttcggcctattggttaaaaaatgagctgatttaacaaaaatttaacgcgaattttaacaaaatattaacgcttacaatttcctgatgcggtattttctccttacgcatctgtgcggtatttcacaccgcatagatcggcaagtgcacaaacaatacttaaataaatactactcagtaataacctatttcttagcatttttgacgaaatttgctattttgttagagtcttttacaccatttgtctccacacctccgcttacatcaacaccaataacgccatttaatctaagcgcatcaccaacattttctggcgtcagtccaccagctaacataaaatgtaagctttcggggctctcttgccttccaacccagtcagaaatcgagttccaatccaaaagttcacctgtcccacctgcttctgaatcaaacaagggaataaacgaatgaggtttctgtgaagctgcactgagtagtatgttgcagtcttttggaaatacgagtcttttaataactggcaaaccgaggaactcttggtattcttgccacgactcatctccatgcagttggacgatatcaatgccgtaatcattgaccagagccaaaacatcctccttaggttgattacgaaacacgccaaccaagtatttcggagtgcctgaactatttttatatgcttttacaagacttgaaattttccttgcaataaccgggtcaattgttctctttctattgggcacacatataatacccagcaagtcagcatcggaatctagagcacattctgcggcctctgtgctctgcaagccgcaaactttcaccaatggaccagaactacctgtgaaattaataacagacatactccaagctgcctttgtgtgcttaatcacgtatactcacgtgctcaatagtcaccaatgccctccctcttggccctctccttttcttttttcgaccgaattaattcttaatcggcaaaaaaagaaaagctccggatcaagattgtacgtaaggtgacaagctatttttcaataaagaatatcttccactactgccatctggcgtcataactgcaaagtacacatatattacgatgctgttctattaaatgcttcctatattatatatatagtaatgtcgtgatctatggtgcactctcagtacaatctgctctgatgccgcatagttaagccagccccgacacccgccaacacccgctgacgcgccctgacgggcttgtctgctcccggcatccgcttacagacaagctgtgaccgtctccgggagctgcatgtgtcagaggttttcaccgtcatcaccgaaacgcgcgagacgaaagggcctcgtgatacgcctatttttataggttaatgtcatgataataatggtttcttagacggatcgcttgcctgtaacttacacgcgcctcgtatcttttaatgatggaataatttgggaatttactctgtgtttatttatttttatgttttgtatttggattttagaaagtaaataaagaaggtagaagagttacggaatgaagaaaaaaaaataaacaaaggtttaaaaaatttcaacaaaaagcgtactttacatatatatttattagacaagaaaagcagattaaatagatatacattcgattaacgataagtaaaatgtaaaatcacaggattttcgtgtgtggtcttctacacagacaagatgaaacaattcggcattaatacctgagagcaggaagagcaagataaaaggtagtatttgttggcgatccccctagagtcttttacatcttcggaaaacaaaaactattttttctttaatttctttttttactttctatttttaatttatatatttatattaaaaaatttaaattataattatttttatagcacgtgatgaaaaggacccaggtggcacttttcggggaaatgtgcgcggaacccctatttgtttatttttctaaatacattcaaatatgtatccgctcatgagacaataaccctgataaatgcttcaataatattgaaaaaggaagagtatgagtattcaacatttccgtgtcgcccttattcccttttttgcggcattttgccttcctgtttttgctcacccagaaacgctggtgaaagtaaaagatgctgaagatcagttgggtgcacgagtgggttacatcgaactggatctcaacagcggtaagatccttgagagttttcgccccgaagaacgttttccaatgatgagcacttttaaagttctgctatgtggcgcggtattatcccgtattgacgccgggcaagagcaactcggtcgccgcatacactattctcagaatgacttggttgagtactcaccagtcacagaaaagcatcttacggatggcatgacagtaagagaattatgcagtgctgccataaccatgagtgataacactgcggccaacttacttctgacaacgatcggaggaccgaaggagctaaccgcttttttgcacaacatgggggatcatgtaactcgccttgatcgttgggaaccggagctgaatgaagccataccaaacgacgagcgtgacaccacgatgcctgtagcaatggcaacaacgttgcgcaaactattaactggcgaactacttactctagcttcccggcaacaattaatagactggatggaggcggataaagttgcaggaccacttctgcgctcggcccttccggctggctggtttattgctgataaatctggagccggtgagcgtgggtctcgcggtatcattgcagcactggggccagatggtaagccctcccgtatcgtagttatctacacgacggggagtcaggcaactatggatgaacgaaatagacagatcgctgagataggtgcctcactgattaagcattggtaactgtcagaccaagtttactcatatatactttagattgatttaaaacttcatttttaatttaaaaggatctaggtgaagatcctttttgataatctcatgaccaaaatcccttaacgtgagttttcgttccactgagcgtcagaccccgtagaaaagatcaaaggatcttcttgagatcctttttttctgcgcgtaatctgctgcttgcaaacaaaaaaaccaccgctaccagcggtggtttgtttgccggatcaagagctaccaactctttttccgaaggtaactggcttcagcagagcgcagataccaaatactgttcttctagtgtagccgtagttaggccaccacttcaagaactctgtagcaccgcctacatacctcgctctgctaatcctgttaccagtggctgctgccagtggcgataagtcgtgtcttaccgggttggactcaagacgatagttaccggataaggcgcagcggtcgggctgaacggggggttcgtgcacacagcccagcttggagcgaacgacctacaccgaactgagatacctacagcgtgagctatgagaaagcgccacgcttcccgaagggagaaaggcggacaggtatccggtaagcggcagggtcggaacaggagagcgcacgagggagcttccagggggaaacgcctggtatctttatagtcctgtcgggtttcgccacctctgacttgagcgtcgatttttgtgatgctcgtcaggggggcggagcctatggaaaaacgccagcaacgcggcctttttacggttcctggccttttgctggccttttgctcacatgttctttcctgcgttatcccctgattctgtggataaccgtattaccgcctttgagtgagctgataccgctcgccgcagccgaacgaccgagcgcagcgagtcagtgagcgaggaagcggaagagcgcccaatacgcaaaccgcctctccccgcgcgttggccgattcattaatgcagctggcacgacaggtttcccgactggaaagcgggcagtgagcgcaacgcaattaatgtgagttagctcactcattaggcaccccaggctttacactttatgcttccggctcgtatgttgtgtggaattgtgagcggataacaatttcacacaggaaacagctatgaccatgattacgccaagctcgaaattaaccctcactaaagggaacaaaagctggtaccaattccttgaattttcaaaaattcttactttttttttggatggacgcaaagaagtttaataatcatattacatggcattaccaccatatacatatccatatctaatcttacttatatgttgtggaaatgtaaagagccccattatcttagcctaaaaaaaccttctctttggaactttcagtaatacgcttaactgctcattgctatattgaagta

SEQ ID NO: 17 - DNA, 6527 bp, synthetic construct
  misc_feature 1..6527: note = Plasmid PW37; note (original language) = Plásmido PW37
  source 1..6527: mol_type = other DNA
cggattagaagccgccgagcgggtgacagccctccgaaggaagactctcctccgtgcgtcctcgtcttcaccggtcgcgttcctgaaacgcagatgtgcctcgcgccgcactgctccgaacaataaagattctacaatactagcttttatggttatgaagaggaaaaattggcagtaacctggccccacaaaccttcaaatgaacgaatcaaattaacaaccataggatgataatgcgattagttttttagccttatttctggggtaattaatcagcgaagcgatgatttttgatctattaacagatatataaatgcaaaaactgcataaccactttaactaatactttcaacattttcggtttgtattacttcttattcaaatgtaataaaagtatcaacaaaaaattgttaatatacctctatactttaacgtcaaggagaaaaaaccccggatcgaattccctacttcatacattttcaattaagatgcagttacttcgctgtttttcaatattttctgttattgcttcagttttagcacaggaactgacaactatatgcgagcaaatcccctcaccaactttagaatcgacgccgtactctttgtcaacgactactattttggccaacgggaaggcaatgcaaggagtttttgaatattacaaatcagtaacgtttgtcagtaattgcggttctcacccctcaacaactagcaaaggcagccccataaacacacagtatgtttttaaggacaatagctcgacgattgaaggtagatacccatacgacgttccagactacgctctgcagttggttccaagaggttctctgcaggctagtggtggaggaggctctggtggaggcggtagcggaggcggagggtcggctagctgcggtggcggcggtactagcaaaatttctcattttttgaaaatggaatctttgaattttattagagctcatactccatatattaatatttacaattgtgaaccagctaatccatctgaaaaaaattctccatctactcaatattgttattctattcaatcttcccaggtcgactgcgggggcggatccgaacaaaagcttatttctgaagaggacttgcaccaccaccaccaccactgactcgagatctgataacaacagtgtagatgtaacaaaatcgactttgttcccactgtacttttagctcgtacaaaatacaatatacttttcatttctccgtaaacaacatgttttcccatgtaatatccttttctatttttcgttccgttaccaactttacacatactttatatagctattcacttctatacactaaaaaactaagacaattttaattttgctgcctgccatatttcaatttgttataaattcctataatttatcctattagtagctaaaaaaagatgaatgtgaatcgaatcctaagagaattgagctccaattcgccctatagtgagtcgtattacaattcactggccgtcgttttacaacgtcgtgactgggaaaaccctggcgttacccaacttaatcgccttgcagcacatccccctttcgccagctggcgtaatagcgaagaggcccgcaccgatcgcctttcccaacagttgcgcagcctgaatggcgaatggacgcgccctgtagcggcgcattaagcgcggcgggtgtggtggttacgcgcagcgtgaccgctacacttgccagcgccctagcgcccgctcctttcgctttcttcccttcctttctcgccacgttcgccggctttccccgtcaagctctaaatcgggggctccctttagggttccgatttagtgctttacggcacctcgaccccaaaaaacttgattagggtgatggttcacgtagtgggccatcgccctgatagacggtttttcgccctttgacgttggagtccacgttctttaatagtggactcttgttccaaactggaacaacactcaaccctatctcggtctattcttttgatttataagggattttgccgatttcggcctattggttaaaaaatgagctgatttaacaaaaatttaacgcgaattttaacaaaatattaacgtttacaatttcctgatgcggtattttctccttacgcatctgtgcggtatttcacaccgcatagatccgtcgagttcaagagaaaaaaaaagaaaaagcaaaaagaaaaaaggaaagcgcgcctcgttcagaatgacacgtatagaatgatgcattaccttgtcatcttcagtatcatactgttcgtatacatacttactgacattcataggtatacatatatacacatgtatatatatcgtatgctgcagctttaaataatcggtgtcactacataagaacacctttggtggagggaacatcgttggtaccattgggcgaggtggcttctcttatggcaaccgcaagagccttgaacgcactctcactacggtgatgatcattcttgcctcgcagacaatcaacgtggagggtaattctgctagcctctgcaaagctttcaagaaaatgcgggatcatctcgcaagagagatctcctactttctccctttgcaaaccaagttcgacaactgcgtacggcctgttcgaaagatctaccaccgctctggaaagtgcctcatccaaaggcgcaaatcctgatccaaacctttttactccacgcgccagtagggcctctttaaaagcttgaccgagagcaatcccgcagtcttcagtggtgtgatggtcgtctatgtgtaagtcaccaatgcactcaacgattagcgaccagccggaatgcttggccagagcatgtatcatatggtccagaaaccctatacctgtgtggacgttaatcacttgcgattgtgtggcctgttctgctactgcttctgcctctttttctgggaagatcgagtgctctatcgctaggggaccaccctttaaagagatcgcaatctgaatcttggtttcatttgtaatacgctttactagggctttctgctctgtcatctttgccttcgtttatcttgcctgctcattttttagtatattcttcgaagaaatcacattactttatataatgtataattcattatgtgataatgccaatcgctaagaaaaaaaaagagtcatccgctaggggaaaaaaaaaaatgaaaatcattaccgaggcataaaaaaatatagagtgtactagaggaggccaagagtaatagaaaaagaaaattgcgggaaaggactgtgttatgacttccctgactaatgccgtgttcaaacgatacctggcagtgactcctagcgctcaccaagctcttaaaacgggaatttatggtgcactctcagtacaatctgctctgatgccgcatagttaagccagccccgacacccgccaacacccgctgacgcgccctgacgggcttgtctgctcccggcatccgcttacagacaagctgtgaccgtctccgggagctgcatgtgtcagaggttttcaccgtcatcaccgaaacgcgcgagacgaaagggcctcgtgatacgcctatttttataggttaatgtcatgataataatggtttcttagacggatcgcttgcctgtaacttacacgcgcctcgtatcttttaatgatggaataatttgggaatttactctgtgtttatttatttttatgttttgtatttggattttagaaagtaaataaagaaggtagaagagttacggaatgaagaaaaaaaaataaacaaaggtttaaaaaatttcaacaaaaagcgtactttacatatatatttattagacaagaaaagcagattaaatagatatacattcgattaacgataagtaaaatgtaaaatcacaggattttcgtgtgtggtcttctacacagacaagatgaaacaattcggcattaatacctgagagcaggaagagcaagataaaaggtagtatttgttggcgatccccctagagtcttttacatcttcggaaaacaaaaactattttttctttaatttctttttttactttctatttttaatttatatatttatattaaaaaatttaaattataattatttttatagcacgtgatgaaaaggacccaggtggcacttttcggggaaatgtgcgcggaacccctatttgtttatttttctaaatacattcaaatatgtatccgctcatgagacaataaccctgataaatgcttcaataatattgaaaaaggaagagtatgagtattcaacatttccgtgtcgcccttattcccttttttgcggcattttgccttcctgtttttgctcacccagaaacgctggtgaaagtaaaagatgctgaagatcagttgggtgcacgagtgggttacatcgaactggatctcaacagcggtaagatccttgagagttttcgccccgaagaacgttttccaatgatgagcacttttaaagttctgctatgtggcgcggtattatcccgtattgacgccgggcaagagcaactcggtcgccgcatacactattctcagaatgacttggttgagtactcaccagtcacagaaaagcatcttacggatggcatgacagtaagagaattatgcagtgctgccataaccatgagtgataacactgcggccaacttacttctgacaacgatcggaggaccgaaggagctaaccgcttttttgcacaacatgggggatcatgtaactcgccttgatcgttgggaaccggagctgaatgaagccataccaaacgacgagcgtgacaccacgatgcctgtagcaatggcaacaacgttgcgcaaactattaactggcgaactacttactctagcttcccggcaacaattaatagactggatggaggcggataaagttgcaggaccacttctgcgctcggcccttccggctggctggtttattgctgataaatctggagccggtgagcgtgggtctcgcggtatcattgcagcactggggccagatggtaagccctcccgtatcgtagttatctacacgacggggagtcaggcaactatggatgaacgaaatagacagatcgctgagataggtgcctcactgattaagcattggtaactgtcagaccaagtttactcatatatactttagattgatttaaaacttcatttttaatttaaaaggatctaggtgaagatcctttttgataatctcatgaccaaaatcccttaacgtgagttttcgttccactgagcgtcagaccccgtagaaaagatcaaaggatcttcttgagatcctttttttctgcgcgtaatctgctgcttgcaaacaaaaaaaccaccgctaccagcggtggtttgtttgccggatcaagagctaccaactctttttccgaaggtaactggcttcagcagagcgcagataccaaatactgttcttctagtgtagccgtagttaggccaccacttcaagaactctgtagcaccgcctacatacctcgctctgctaatcctgttaccagtggctgctgccagtggcgataagtcgtgtcttaccgggttggactcaagacgatagttaccggataaggcgcagcggtcgggctgaacggggggttcgtgcacacagcccagcttggagcgaacgacctacaccgaactgagatacctacagcgtgagctatgagaaagcgccacgcttcccgaagggagaaaggcggacaggtatccggtaagcggcagggtcggaacaggagagcgcacgagggagcttccagggggaaacgcctggtatctttatagtcctgtcgggtttcgccacctctgacttgagcgtcgatttttgtgatgctcgtcaggggggcggagcctatggaaaaacgccagcaacgcggcctttttacggttcctggccttttgctggccttttgctcacatgttctttcctgcgttatcccctgattctgtggataaccgtattaccgcctttgagtgagctgataccgctcgccgcagccgaacgaccgagcgcagcgagtcagtgagcgaggaagcggaagagcgcccaatacgcaaaccgcctctccccgcgcgttggccgattcattaatgcagctggcacgacaggtttcccgactggaaagcgggcagtgagcgcaacgcaattaatgtgagttagctcactcattaggcaccccaggctttacactttatgcttccggctcgtatgttgtgtggaattgtgagcggataacaatttcacacaggaaacagctatgaccatgattacgccaagctcgaaattaaccctcactaaagggaacaaaagctggtaccaattccttgaattttcaaaaattcttactttttttttggatggacgcaaagaagtttaataatcatattacatggcattaccaccatatacatatccatatctaatcttacttatatgttgtggaaatgtaaagagccccattatcttagcctaaaaaaaccttctctttggaactttcagtaatacgcttaactgctcattgctatattgaagta

SEQ ID NO: 18 - DNA, 7571 bp, synthetic construct
  misc_feature 1..7571: note = Plasmid PW38; note (original language) = Plásmido PW38
  source 1..7571: mol_type = other DNA
cggattagaagccgccgagcgggtgacagccctccgaaggaagactctcctccgtgcgtcctcgtcttcaccggtcgcgttcctgaaacgcagatgtgcctcgcgccgcactgctccgaacaataaagattctacaatactagcttttatggttatgaagaggaaaaattggcagtaacctggccccacaaaccttcaaatgaacgaatcaaattaacaaccataggatgataatgcgattagttttttagccttatttctggggtaattaatcagcgaagcgatgatttttgatctattaacagatatataaatgcaaaaactgcataaccactttaactaatactttcaacattttcggtttgtattacttcttattcaaatgtaataaaagtatcaacaaaaaattgttaatatacctctatactttaacgtcaaggagaaaaaaccccggatcgaattccctacttcatacattttcaattaagatgcagttacttcgctgtttttcaatattttctgttattgcttcagttttagcacaggaactgacaactatatgcgagcaaatcccctcaccaactttagaatcgacgccgtactctttgtcaacgactactattttggccaacgggaaggcaatgcaaggagtttttgaatattacaaatcagtaacgtttgtcagtaattgcggttctcacccctcaacaactagcaaaggcagccccataaacacacagtatgtttttaaggacaatagctcgacgattgaaggtagatacccatacgacgttccagactacgctctgcagttggttccaagaggttctctgcaggctagtggtggaggaggctctggtggaggcggtagcggaggcggagggtcggctagctgcggtggcggcggtactagcaaaatttctcattttttgaaaatggaatctttgaattttattagagctcatactccatatattaatatttacaattgtgaaccagctaatccatctgaaaaaaattctccatctactcaatattgttattctattcaatcttcccaggtcgactgcgggggcggatccgaacaaaagcttatttctgaagaggacttgcaccaccaccaccaccactgactcgagatctgataacaacagtgtagatgtaacaaaatcgactttgttcccactgtacttttagctcgtacaaaatacaatatacttttcatttctccgtaaacaacatgttttcccatgtaatatccttttctatttttcgttccgttaccaactttacacatactttatatagctattcacttctatacactaaaaaactaagacaattttaattttgctgcctgccatatttcaatttgttataaattcctataatttatcctattagtagctaaaaaaagatgaatgtgaatcgaatcctaagagaattgagctccaattcgccctatagtgagtcgtattacaattcactggccgtcgttttacaacgtcgtgactgggaaaaccctggcgttacccaacttaatcgccttgcagcacatccccctttcgccagctggcgtaatagcgaagaggcccgcaccgatcgcctttcccaacagttgcgcagcctgaatggcgaatggacgcgccctgtagcggcgcattaagcgcggcgggtgtggtggttacgcgcagcgtgaccgctacacttgccagcgccctagcgcccgctcctttcgctttcttcccttcctttctcgccacgttcgccggctttccccgtcaagctctaaatcgggggctccctttagggttccgatttagtgctttacggcacctcgaccccaaaaaacttgattagggtgatggttcacgtagtgggccatcgccctgatagacggtttttcgccctttgacgttggagtccacgttctttaatagtggactcttgttccaaactggaacaacactcaaccctatctcggtctattcttttgatttataagggattttgccgatttcggcctattggttaaaaaatgagctgatttaacaaaaatttaacgcgaattttaacaaaatattaacgcttacaatttcctgatgcggtattttctccttacgcatctgtgcggtatttcacaccgcatatcgaccggtcgaggagaacttctagtatatctacatacctaatattattgccttattaaaaatggaatcccaacaattacatcaaaatccacattctcttcaaaatcaattgtcctgtacttccttgttcatgtgtgttcaaaaacgttatatttataggataattatactctatttctcaacaagtaattggttgtttggccgagcggtctaaggcgcctgattcaagaaatatcttgaccgcagttaactgtgggaatactcaggtatcgtaagatgcaagagttcgaatctcttagcaaccattatttttttcctcaacataacgagaacacacaggggcgctatcgcacagaatcaaattcgatgactggaaattttttgttaatttcagaggtcgcctgacgcatatacctttttcaactgaaaaattgggagaaaaaggaaaggtgagagcgccggaaccggcttttcatatagaatagagaagcgttcatgactaaatgcttgcatcacaatacttgaagttgacaatattatttaaggacctattgttttttccaataggtggttagcaatcgtcttactttctaacttttcttaccttttacatttcagcaatatatatatatatatttcaaggatataccattctaatgtctgcccctaagaagatcgtcgttttgccaggtgaccacgttggtcaagaaatcacagccgaagccattaaggttcttaaagctatttctgatgttcgttccaatgtcaagttcgatttcgaaaatcatttaattggtggtgctgctatcgatgctacaggtgttccacttccagatgaggcgctggaagcctccaagaaggctgatgccgttttgttaggtgctgtgggtggtcctaaatggggtaccggtagtgttagacctgaacaaggtttactaaaaatccgtaaagaacttcaattgtacgccaacttaagaccatgtaactttgcatccgactctcttttagacttatctccaatcaagccacaatttgctaaaggtactgacttcgttgttgtcagagaattagtgggaggtatttactttggtaagagaaaggaagacgatggtgatggtgtcgcttgggatagtgaacaatacaccgttccagaagtgcaaagaatcacaagaatggccgctttcatggccctacaacatgagccaccattgcctatttggtccttggataaagctaatgttttggcctcttcaagattatggagaaaaactgtggaggaaaccatcaagaacgaattccctacattgaaggttcaacatcaattgattgattctgccgccatgatcctagttaagaacccaacccacctaaatggtattataatcaccagcaacatgtttggtgatatcatctccgatgaagcctccgttatcccaggttccttgggtttgttgccatctgcgtccttggcctctttgccagacaagaacaccgcatttggtttgtacgaaccatgccacggttctgctccagatttgccaaagaataaggtcaaccctatcgccactatcttgtctgctgcaatgatgttgaaattgtcattgaacttgcctgaagaaggtaaggccattgaagatgcagttaaaaaggttttggatgcaggtatcagaactggtgatttaggtggttccaacagtaccaccgaagtcggtgatgctgtcgccgaagaagttaagaaaatccttgcttaaaaagattctctttttttatgatatttgtacataaactttataaatgaaattcataatagaaacgacacgaaattacaaaatggaatatgttcatagggtagacgaaactatatacgcaatctacatacatttatcaagaaggagaaaaaggaggatgtaaaggaatacaggtaagcaaattgatactaatggctcaacgtgataaggaaaaagaattgcactttaacattaatattgacaaggaggagggcaccacacaaaaagttaggtgtaacagaaaatcatgaaactatgattcctaatttatatattggaggattttctctaaaaaaaaaaaaatacaacaaataaaaaacactcaatgacctgaccatttgatggagtttaagtcaataccttcttgaaccatttcccataatggtgaaagttccctcaagaattttactctgtcagaaacggccttaacgacgtagtcgatatggtgcactctcagtacaatctgctctgatgccgcatagttaagccagccccgacacccgccaacacccgctgacgcgccctgacgggcttgtctgctcccggcatccgcttacagacaagctgtgaccgtctccgggagctgcatgtgtcagaggttttcaccgtcatcaccgaaacgcgcgagacgaaagggcctcgtgatacgcctatttttataggttaatgtcatgataataatggtttcttagacggatcgcttgcctgtaacttacacgcgcctcgtatcttttaatgatggaataatttgggaatttactctgtgtttatttatttttatgttttgtatttggattttagaaagtaaataaagaaggtagaagagttacggaatgaagaaaaaaaaataaacaaaggtttaaaaaatttcaacaaaaagcgtactttacatatatatttattagacaagaaaagcagattaaatagatatacattcgattaacgataagtaaaatgtaaaatcacaggattttcgtgtgtggtcttctacacagacaagatgaaacaattcggcattaatacctgagagcaggaagagcaagataaaaggtagtatttgttggcgatccccctagagtcttttacatcttcggaaaacaaaaactattttttctttaatttctttttttactttctatttttaatttatatatttatattaaaaaatttaaattataattatttttatagcacgtgatgaaaaggacccaggtggcacttttcggggaaatgtgcgcggaacccctatttgtttatttttctaaatacattcaaatatgtatccgctcatgagacaataaccctgataaatgcttcaataatattgaaaaaggaagagtatgagtattcaacatttccgtgtcgcccttattcccttttttgcggcattttgccttcctgtttttgctcacccagaaacgctggtgaaagtaaaagatgctgaagatcagttgggtgcacgagtgggttacatcgaactggatctcaacagcggtaagatccttgagagttttcgccccgaagaacgttttccaatgatgagcacttttaaagttctgctatgtggcgcggtattatcccgtattgacgccgggcaagagcaactcggtcgccgcatacactattctcagaatgacttggttgagtactcaccagtcacagaaaagcatcttacggatggcatgacagtaagagaattatgcagtgctgccataaccatgagtgataacactgcggccaacttacttctgacaacgatcggaggaccgaaggagctaaccgcttttttgcacaacatgggggatcatgtaactcgccttgatcgttgggaaccggagctgaatgaagccataccaaacgacgagcgtgacaccacgatgcctgtagcaatggcaacaacgttgcgcaaactattaactggcgaactacttactctagcttcccggcaacaattaatagactggatggaggcggataaagttgcaggaccacttctgcgctcggcccttccggctggctggtttattgctgataaatctggagccggtgagcgtgggtctcgcggtatcattgcagcactggggccagatggtaagccctcccgtatcgtagttatctacacgacggggagtcaggcaactatggatgaacgaaatagacagatcgctgagataggtgcctcactgattaagcattggtaactgtcagaccaagtttactcatatatactttagattgatttaaaacttcatttttaatttaaaaggatctaggtgaagatcctttttgataatctcatgaccaaaatcccttaacgtgagttttcgttccactgagcgtcagaccccgtagaaaagatcaaaggatcttcttgagatcctttttttctgcgcgtaatctgctgcttgcaaacaaaaaaaccaccgctaccagcggtggtttgtttgccggatcaagagctaccaactctttttccgaaggtaactggcttcagcagagcgcagataccaaatactgttcttctagtgtagccgtagttaggccaccacttcaagaactctgtagcaccgcctacatacctcgctctgctaatcctgttaccagtggctgctgccagtggcgataagtcgtgtcttaccgggttggactcaagacgatagttaccggataaggcgcagcggtcgggctgaacggggggttcgtgcacacagcccagcttggagcgaacgacctacaccgaactgagatacctacagcgtgagctatgagaaagcgccacgcttcccgaagggagaaaggcggacaggtatccggtaagcggcagggtcggaacaggagagcgcacgagggagcttccagggggaaacgcctggtatctttatagtcctgtcgggtttcgccacctctgacttgagcgtcgatttttgtgatgctcgtcaggggggcggagcctatggaaaaacgccagcaacgcggcctttttacggttcctggccttttgctggccttttgctcacatgttctttcctgcgttatcccctgattctgtggataaccgtattaccgcctttgagtgagctgataccgctcgccgcagccgaacgaccgagcgcagcgagtcagtgagcgaggaagcggaagagcgcccaatacgcaaaccgcctctccccgcgcgttggccgattcattaatgcagctggcacgacaggtttcccgactggaaagcgggcagtgagcgcaacgcaattaatgtgagttagctcactcattaggcaccccaggctttacactttatgcttccggctcgtatgttgtgtggaattgtgagcggataacaatttcacacaggaaacagctatgaccatgattacgccaagctcgaaattaaccctcactaaagggaacaaaagctggtaccaattccttgaattttcaaaaattcttactttttttttggatggacgcaaagaagtttaataatcatattacatggcattaccaccatatacatatccatatctaatcttacttatatgttgtggaaatgtaaagagccccattatcttagcctaaaaaaaccttctctttggaactttcagtaatacgcttaactgctcattgctatattgaagta

SEQ ID NO: 19 - DNA, 6314 bp, synthetic construct
  misc_feature 1..6314: note = Plasmid pCTcon2; note (original language) = Plásmido pCTcon2
  source 1..6314: mol_type = other DNA
cggattagaagccgccgagcgggtgacagccctccgaaggaagactctcctccgtgcgtcctcgtcttcaccggtcgcgttcctgaaacgcagatgtgcctcgcgccgcactgctccgaacaataaagattctacaatactagcttttatggttatgaagaggaaaaattggcagtaacctggccccacaaaccttcaaatgaacgaatcaaattaacaaccataggatgataatgcgattagttttttagccttatttctggggtaattaatcagcgaagcgatgatttttgatctattaacagatatataaatgcaaaaactgcataaccactttaactaatactttcaacattttcggtttgtattacttcttattcaaatgtaataaaagtatcaacaaaaaattgttaatatacctctatactttaacgtcaaggagaaaaaaccccggatcgaattccctacttcatacattttcaattaagatgcagttacttcgctgtttttcaatattttctgttattgcttcagttttagcacaggaactgacaactatatgcgagcaaatcccctcaccaactttagaatcgacgccgtactctttgtcaacgactactattttggccaacgggaaggcaatgcaaggagtttttgaatattacaaatcagtaacgtttgtcagtaattgcggttctcacccctcaacaactagcaaaggcagccccataaacacacagtatgtttttaaggacaatagctcgacgattgaaggtagatacccatacgacgttccagactacgctctgcaggctagtggtggaggaggctctggtggaggcggtagcggaggcggagggtcggctagctgcggtggcggcggtactagcaaaatttctcattttttgaaaatggaatctttgaattttattagagctcatactccatatattaatatttacaattgtgaaccagctaatccatctgaaaaaaattctccatctactcaatattgttattctattcaatcttcccaggtcgactgcgggggcggatccgaacaaaagcttatttctgaagaggacttgtaatagctcgagatctgataacaacagtgtagatgtaacaaaatcgactttgttcccactgtacttttagctcgtacaaaatacaatatacttttcatttctccgtaaacaacatgttttcccatgtaatatccttttctatttttcgttccgttaccaactttacacatactttatatagctattcacttctatacactaaaaaactaagacaattttaattttgctgcctgccatatttcaatttgttataaattcctataatttatcctattagtagctaaaaaaagatgaatgtgaatcgaatcctaagagaattgagctccaattcgccctatagtgagtcgtattacaattcactggccgtcgttttacaacgtcgtgactgggaaaaccctggcgttacccaacttaatcgccttgcagcacatccccctttcgccagctggcgtaatagcgaagaggcccgcaccgatcgcctttcccaacagttgcgcagcctgaatggcgaatggacgcgccctgtagcggcgcattaagcgcggcgggtgtggtggttacgcgcagcgtgaccgctacacttgccagcgccctagcgcccgctcctttcgctttcttcccttcctttctcgccacgttcgccggctttccccgtcaagctctaaatcgggggctccctttagggttccgatttagtgctttacggcacctcgaccccaaaaaacttgattagggtgatggttcacgtagtgggccatcgccctgatagacggtttttcgccctttgacgttggagtccacgttctttaatagtggactcttgttccaaactggaacaacactcaaccctatctcggtctattcttttgatttataagggattttgccgatttcggcctattggttaaaaaatgagctgatttaacaaaaatttaacgcgaattttaacaaaatattaacgcttacaatttcctgatgcggtattttctccttacgcatctgtgcggtatttcacaccgcatagatcggcaagtgcacaaacaatacttaaataaatactactcagtaataacctatttcttagcatttttgacgaaatttgctattttgttagagtcttttacaccatttgtctccacacctccgcttacatcaacaccaataacgccatttaatctaagcgcatcaccaacattttctggcgtcagtccaccagctaacataaaatgtaagctttcggggctctcttgccttccaacccagtcagaaatcgagttccaatccaaaagttcacctgtcccacctgcttctgaatcaaacaagggaataaacgaatgaggtttctgtgaagctgcactgagtagtatgttgcagtcttttggaaatacgagtcttttaataactggcaaaccgaggaactcttggtattcttgccacgactcatctccatgcagttggacgatatcaatgccgtaatcattgaccagagccaaaacatcctccttaggttgattacgaaacacgccaaccaagtatttcggagtgcctgaactatttttatatgcttttacaagacttgaaattttccttgcaataaccgggtcaattgttctctttctattgggcacacatataatacccagcaagtcagcatcggaatctagagcacattctgcggcctctgtgctctgcaagccgcaaactttcaccaatggaccagaactacctgtgaaattaataacagacatactccaagctgcctttgtgtgcttaatcacgtatactcacgtgctcaatagtcaccaatgccctccctcttggccctctccttttcttttttcgaccgaattaattcttaatcggcaaaaaaagaaaagctccggatcaagattgtacgtaaggtgacaagctatttttcaataaagaatatcttccactactgccatctggcgtcataactgcaaagtacacatatattacgatgctgttctattaaatgcttcctatattatatatatagtaatgtcgtgatctatggtgcactctcagtacaatctgctctgatgccgcatagttaagccagccccgacacccgccaacacccgctgacgcgccctgacgggcttgtctgctcccggcatccgcttacagacaagctgtgaccgtctccgggagctgcatgtgtcagaggttttcaccgtcatcaccgaaacgcgcgagacgaaagggcctcgtgatacgcctatttttataggttaatgtcatgataataatggtttcttagacggatcgcttgcctgtaacttacacgcgcctcgtatcttttaatgatggaataatttgggaatttactctgtgtttatttatttttatgttttgtatttggattttagaaagtaaataaagaaggtagaagagttacggaatgaagaaaaaaaaataaacaaaggtttaaaaaatttcaacaaaaagcgtactttacatatatatttattagacaagaaaagcagattaaatagatatacattcgattaacgataagtaaaatgtaaaatcacaggattttcgtgtgtggtcttctacacagacaagatgaaacaattcggcattaatacctgagagcaggaagagcaagataaaaggtagtatttgttggcgatccccctagagtcttttacatcttcggaaaacaaaaactattttttctttaatttctttttttactttctatttttaatttatatatttatattaaaaaatttaaattataattatttttatagcacgtgatgaaaaggacccaggtggcacttttcggggaaatgtgcgcggaacccctatttgtttatttttctaaatacattcaaatatgtatccgctcatgagacaataaccctgataaatgcttcaataatattgaaaaaggaagagtatgagtattcaacatttccgtgtcgcccttattcccttttttgcggcattttgccttcctgtttttgctcacccagaaacgctggtgaaagtaaaagatgctgaagatcagttgggtgcacgagtgggttacatcgaactggatctcaacagcggtaagatccttgagagttttcgccccgaagaacgttttccaatgatgagcacttttaaagttctgctatgtggcgcggtattatcccgtattgacgccgggcaagagcaactcggtcgccgcatacactattctcagaatgacttggttgagtactcaccagtcacagaaaagcatcttacggatggcatgacagtaagagaattatgcagtgctgccataaccatgagtgataacactgcggccaacttacttctgacaacgatcggaggaccgaaggagctaaccgcttttttgcacaacatgggggatcatgtaactcgccttgatcgttgggaaccggagctgaatgaagccataccaaacgacgagcgtgacaccacgatgcctgtagcaatggcaacaacgttgcgcaaactattaactggcgaactacttactctagcttcccggcaacaattaatagactggatggaggcggataaagttgcaggaccacttctgcgctcggcccttccggctggctggtttattgctgataaatctggagccggtgagcgtgggtctcgcggtatcattgcagcactggggccagatggtaagccctcccgtatcgtagttatctacacgacggggagtcaggcaactatggatgaacgaaatagacagatcgctgagataggtgcctcactgattaagcattggtaactgtcagaccaagtttactcatatatactttagattgatttaaaacttcatttttaatttaaaaggatctaggtgaagatcctttttgataatctcatgaccaaaatcccttaacgtgagttttcgttccactgagcgtcagaccccgtagaaaagatcaaaggatcttcttgagatcctttttttctgcgcgtaatctgctgcttgcaaacaaaaaaaccaccgctaccagcggtggtttgtttgccggatcaagagctaccaactctttttccgaaggtaactggcttcagcagagcgcagataccaaatactgttcttctagtgtagccgtagttaggccaccacttcaagaactctgtagcaccgcctacatacctcgctctgctaatcctgttaccagtggctgctgccagtggcgataagtcgtgtcttaccgggttggactcaagacgatagttaccggataaggcgcagcggtcgggctgaacggggggttcgtgcacacagcccagcttggagcgaacgacctacaccgaactgagatacctacagcgtgagctatgagaaagcgccacgcttcccgaagggagaaaggcggacaggtatccggtaagcggcagggtcggaacaggagagcgcacgagggagcttccagggggaaacgcctggtatctttatagtcctgtcgggtttcgccacctctgacttgagcgtcgatttttgtgatgctcgtcaggggggcggagcctatggaaaaacgccagcaacgcggcctttttacggttcctggccttttgctggccttttgctcacatgttctttcctgcgttatcccctgattctgtggataaccgtattaccgcctttgagtgagctgataccgctcgccgcagccgaacgaccgagcgcagcgagtcagtgagcgaggaagcggaagagcgcccaatacgcaaaccgcctctccccgcgcgttggccgattcattaatgcagctggcacgacaggtttcccgactggaaagcgggcagtgagcgcaacgcaattaatgtgagttagctcactcattaggcaccccaggctttacactttatgcttccggctcgtatgttgtgtggaattgtgagcggataacaatttcacacaggaaacagctatgaccatgattacgccaagctcgaaattaaccctcactaaagggaacaaaagctggtaccaattccttgaattttcaaaaattcttactttttttttggatggacgcaaagaagtttaataatcatattacatggcattaccaccatatacatatccatatctaatcttacttatatgttgtggaaatgtaaagagccccattatcttagcctaaaaaaaccttctctttggaactttcagtaatacgcttaactgctcattgctatattgaagta

SEQ ID NO: 20 - DNA, 2178 bp, Saccharomyces cerevisiae
  source 1..2178: mol_type = genomic DNA
atgacattatctttcgctcattttacctacctgttcacaatattgttgggattaactaatattgccttggcatctgatccagaaacgattctagtgacgataaccaagacaaacgatgcaaatggggttgttacaactacagtttcacccgcgctagtctccacatccactatcgttcaagctggcactacgacattgtatacgacttggtgtccattgacggtatccacttcatctgctgccgaaataagtccttcaatatcgtacgctactaccctatccagatttagtactttgacattatctacagaagtctgctcccatgaggcatgtccttcgtcatcgacgttgccaaccaccaccttatctgtgacttccaagttcacttcatatatttgccctacttgtcacacaaccgctatcagctcattatccgaagtaggaactacaaccgtggtatcatccagcgccattgaaccatcaagtgcctctataatctcacctgtcacctctacactttcgagtacaacatcgtccaatccaactactacctccctaagttcgacatctacatctccaagctctacatctacatctccaagctctacatctacctcatcaagttcgacatctacctcatcaagttcgacatctacctcatcaagttcgacatctacatctccaagttcgacatccacatcttcaagtttgacatccacatcttcaagttctacatctacatcccaaagttctacatctacctcatcaagttcgacatctacatctccaagctctacatctacctcatcaagttcaacatctacatctccaagttctaaatctacttctgcaagctccacttccacttcttcatattcaacatctacatccccaagtttgacttcttcatctccaactttggcttccacttctccaagttcaacatctattagctctacttttactgattcaacttcatcccttggctcctctatagcatcttcatcaacgtctgtgtcattatacagcccatccacacctgtttactccgtcccttcgacttcgtcaaatgttgcaactccttctatgacttcttcaactgttgaaacaactgttagttcacaaagttcgtctgaatatatcaccaaatcctcaatttctactactatcccatcattttccatgtctacatatttcaccactgttagtggagtcactacaatgtatacgacatggtgtccttatagctctgaatctgagactagcacattaaccagtatgcatgaaacggttacaacagacgctacagtctgcactcacgagtcttgcatgccctcgcagacaacaagtttgattacatcttctataaaaatgtccactaaaaacgtcgcaacttctgtaagcacctcaacggttgaatcctcatatgcatgctccacatgtgctgaaacgtcacactcgtattcttccgtgcaaacagcttcatcaagttctgtaacacagcagaccacatccacaaagagttgggtaagttcaatgacaacttcggatgaagatttcaataagcacgctaccggtaagtatcatgtaacatcttcaggtacctcaaccatttcgactagtgtaagtgaagccacgagtacatcaagcattgactcagaatctcaagaacaatcatcacacttattatcgacatcggtcctttcatcctcctccttgtctgctacattatcctctgacagtactattttgctattcagttctgtatcatcactaagtgtcgaacagtcaccagttaccacacttcaaatttcttcaacatcagagattttacaacccacttcttccacagctattgctacaatatctgcctctacatcatcactttccgcaacatctatctctacaccatctacctctgtggaatcgactattgaatcttcatcattgactccgacggtatcttctattttcctctcatcatcatctgctccctcttctctacaaacatctgttaccactacagaagtttccactacttcaatctccatacaataccaaacttcatcaatggtaacaattagccaatatatgggcagtggatcgcaaacgcgtttgccattaggaaagttggtcttcgccatcatggcagttgcttgcaatgtaattttcagttaa

SEQ ID NO: 21 - DNA, 71 bp, synthetic construct
  misc_feature 1..71: note = Primer GAL1-AGA1 Fw; note (original language) = Cebador GAL1-AGA1 Fw
  source 1..71: mol_type = other DNA
ggatattgcacgtttcaagtcaaaacgcggctgtaacataattttcgcggcatcagagcagattgtactga

SEQ ID NO: 22 - DNA, 71 bp, synthetic construct
  misc_feature 1..71: note = Primer GAL1-AGA1 Rv; note (original language) = Cebador GAL1-AGA1 Rv
  source 1..71: mol_type = other DNA
caatattgtgaacaggtaggtaaaatgagcgaaagataatgtcatgggggatccactagttctagaatccg

SEQ ID NO: 23 - DNA, 22 bp, synthetic construct
  misc_feature 1..22: note = Oligonucleotide F1ori1-F; note (original language) = Oligonucleótido F1ori1-F
  source 1..22: mol_type = other DNA
gtggactcttgttccaaactgg

SEQ ID NO: 24 - DNA, 20 bp, synthetic construct
  misc_feature 1..20: note = Oligonucleotide PRS-marker; note (original language) = Oligonucleótido PRS-marker
  source 1..20: mol_type = other DNA
cggcatcagagcagattgta

SEQ ID NO: 25 - DNA, 41 bp, synthetic construct
  misc_feature 1..41: note = Oligonucleotide TEV Fw; note (original language) = Oligonucleótido TEV Fw
  source 1..41: mol_type = other DNA
ccccctgcaggaaaatttgtattttcaatctctgcaggggg

SEQ ID NO: 26 - DNA, 41 bp, synthetic construct
  misc_feature 1..41: note = Oligonucleotide TEV Rev; note (original language) = Oligonucleótido TEV Rev
  source 1..41: mol_type = other DNA
ccccctgcagagattgaaaatacaaattttcctgcaggggg

SEQ ID NO: 27 - DNA, 38 bp, synthetic construct
  misc_feature 1..38: note = Oligonucleotide THROMBIN Fw; note (original language) = Oligonucleótido THROMBIN Fw
  source 1..38: mol_type = other DNA
ccccctgcagttggttccaagaggttctctgcaggggg

SEQ ID NO: 28 - DNA, 38 bp, synthetic construct
  misc_feature 1..38: note = Oligonucleotide THROMBIN Rv; note (original language) = Oligonucleótido THROMBIN Rv
  source 1..38: mol_type = other DNA
ccccctgcagagaacctcttggaaccaactgcaggggg

SEQ ID NO: 29 - DNA, 83 bp, synthetic construct
  misc_feature 1..83: note = Oligonucleotide HISF; note (original language) = Oligonucleótido HISF
  source 1..83: mol_type = other DNA
gaacaaaagcttatttctgaagaggacttgcaccaccaccaccaccactgactcgagatctgataacaacagtgtagatgtaa

SEQ ID NO: 30 - DNA, 83 bp, synthetic construct
  misc_feature 1..83: note = Oligonucleotide HISR; note (original language) = Oligonucleótido HISR
  source 1..83: mol_type = other DNA
ttacatctacactgttgttatcagatctcgagtcagtggtggtggtggtggtgcaagtcctcttcagaaataagcttttgttc

SEQ ID NO: 31 - protein, 87 aa, Saccharomyces cerevisiae
MQLLRCFSIFSVIASVLAQELTTICEQIPSPTLESTPYSLSTTTILANGKAMQGVFEYYKSVTFVSNCGSHPSTTSKGSPINTQYVF

SEQ ID NO: 32 - protein, 8 aa, synthetic construct
  REGION 1..8: note = Tag DYKDDDDK; note (original language) = Etiqueta DYKDDDDK
DYKDDDDK

SEQ ID NO: 33 - protein, 10 aa, synthetic construct
  REGION 1..10: note = Tag Glu-Glu; note (original language) = Etiqueta Glu-Glu
CEEEEYMPME

SEQ ID NO: 34 - protein, 8 aa, synthetic construct
  REGION 1..8: note = Tag Strep-Tag; note (original language) = Etiqueta Strep-Tag
WRHPQFGG

SEQ ID NO: 35 - protein, 4 aa, synthetic construct
  REGION 1..4: note = Tag VSV-G; note (original language) = Etiqueta VSV-G
VSVG

SEQ ID NO: 36 - protein, 7 aa, synthetic construct
  REGION 1..7: note = TEV proteasa excision sequence; note (original language) = Secuencia de escisión de la proteasa TEV
ENLYFQG

SEQ ID NO: 37 - protein, 5 aa, synthetic construct
  REGION 1..5: note = HRV3C protease excision sequence; note (original language) = Secuencia de escisión de la proteasa HRV3C
LFQGP

SEQ ID NO: 38 - protein, 6 aa, synthetic construct
  REGION 1..6: note = Thrombin protease excision sequence; note (original language) = Secuencia de escisión de la proteasa Trombina
LVPRGS

SEQ ID NO: 39 - protein, 4 aa, synthetic construct
  REGION 1..4: note = FactorXA protease excision sequence; note (original language) = Secuencia de escisión de la proteasa FactorXA
  VARIANT 2: note = E may be replaced with D; note (original language) = E puede ser sustituida por D
IEGR

SEQ ID NO: 40 - protein, 5 aa, synthetic construct
  REGION 1..5: note = Enterokinase protease excision sequence; note (original language) = Secuencia de escisión de la proteasa enteroquinasa
DDDDK